European Patent Specification EP 3 344 660 B1, published March 5, 2025. Title: TGF-Beta Receptor Ectodomain Fusion Molecules and Uses Thereof. Applicant: National Research Council of Canada O'Connor, Maureen Sulea, Traian Zwaagstra, John C. Jaramillo, Maria  C. Lenferink, Anne E.G. The sequence listing filed with the application follows.

SEQUENCE LISTING (150 sequences)

SEQ ID NO: 1 - protein, 217 aa, Artificial Sequence
  Human IgG1 Fc region
APELLGGPSVFLFPPKPKDTLMISRTPEVTCVVVDVSHEDPEVKFNWYVDGVEVHNAKTKPREEQYNSTYRVVSVLTVLHQDWLNGKEYKCKVSNKALPAPIEKTISKAKGQPREPQVYTLPPSRDELTKNQVSLTCLVKGFYPSDIAVEWESNGQPENNYKTTPPVLDSDGSFFLYSKLTVDKSRWQQGNVFSCSVMHEALHNHYTQKSLSLSPGK

SEQ ID NO: 2 - protein, 216 aa, Artificial Sequence
  Human IgG2 Fc region
APPVAGPSVFLFPPKPKDTLMISRTPEVTCVVVDVSHEDPEVQFNWYVDGVEVHNAKTKPREEQFNSTFRVVSVLTVVHQDWLNGKEYKCKVSNKGLPAPIEKTISKTKGQPREPQVYTLPPSREEMTKNQVSLTCLVKGFYPSDISVEWESNGQPENNYKTTPPMLDSDGSFFLYSKLTVDKSRWQQGNVFSCSVMHEALHNHYTQKSLSLSPGK

SEQ ID NO: 3 - protein, 217 aa, Artificial Sequence
  Human IgG3 Fc region
APELLGGPSVFLFPPKPKDTLMISRTPEVTCVVVDVSHEDPEVQFKWYVDGVEVHNAKTKPREEQYNSTFRVVSVLTVLHQDWLNGKEYKCKVSNKALPAPIEKTISKTKGQPREPQVYTLPPSREEMTKNQVSLTCLVKGFYPSDIAVEWESSGQPENNYNTTPPMLDSDGSFFLYSKLTVDKSRWQQGNIFSCSVMHEALHNRFTQKSLSLSPGK

SEQ ID NO: 4 - protein, 217 aa, Artificial Sequence
  Human IgG4 Fc region
APEFLGGPSVFLFPPKPKDTLMISRTPEVTCVVVDVSQEDPEVQFNWYVDGVEVHNAKTKPREEQFNSTYRVVSVLTVLHQDWLNGKEYKCKVSNKGLPSSIEKTISKAKGQPREPQVYTLPPSQEEMTKNQVSLTCLVKGFYPSDIAVEWESNGQPENNYKTTPPVLDSDGSFFLYSRLTVDKSRWQEGNVFSCSVMHEALHNHYTQKSLSLSLGK

SEQ ID NO: 5 - protein, 15 aa, Artificial Sequence
  Human IgG1 hinge region
EPKSCDKTHTCPPCP

SEQ ID NO: 6 - protein, 12 aa, Artificial Sequence
  Human IgG2 hinge region
ERKCCVECPPCP

SEQ ID NO: 7 - protein, 62 aa, Artificial Sequence
  Human IgG3 hinge region
ELKTPLGDTTHTCPRCPEPKSCDTPPPCPRCPEPKSCDTPPPCPRCPEPKSCDTPPPCPRCP

SEQ ID NO: 8 - protein, 12 aa, Artificial Sequence
  Human IgG4 hinge region
ESKYGPPCPSCP

SEQ ID NO: 9 - protein, 216 aa, Artificial Sequence
  hIgG1FcdeltaK-deltaC Fc variant
APELLGGPSVFLFPPKPKDTLMISRTPEVTCVVVDVSHEDPEVKFNWYVDGVEVHNAKTKPREEQYNSTYRVVSVLTVLHQDWLNGKEYKCKVSNKALPAPIEKTISKAKGQPREPQVYTLPPSRDELTKNQVSLTCLVKGFYPSDIAVEWESNGQPENNYKTTPPVLDSDGSFFLYSKLTVDKSRWQQGNVFSCSVMHEALHNHYTQKSLSLSPG

SEQ ID NO: 10 - protein, 220 aa, Artificial Sequence
  hIgG1FcdeltaK-C Fc variant
PPCPAPELLGGPSVFLFPPKPKDTLMISRTPEVTCVVVDVSHEDPEVKFNWYVDGVEVHNAKTKPREEQYNSTYRVVSVLTVLHQDWLNGKEYKCKVSNKALPAPIEKTISKAKGQPREPQVYTLPPSRDELTKNQVSLTCLVKGFYPSDIAVEWESNGQPENNYKTTPPVLDSDGSFFLYSKLTVDKSRWQQGNVFSCSVMHEALHNHYTQKSLSLSPG

SEQ ID NO: 11 - protein, 226 aa, Artificial Sequence
  hIgG1FcdeltaK-CC Fc variant
DKTHTCPPCPAPELLGGPSVFLFPPKPKDTLMISRTPEVTCVVVDVSHEDPEVKFNWYVDGVEVHNAKTKPREEQYNSTYRVVSVLTVLHQDWLNGKEYKCKVSNKALPAPIEKTISKAKGQPREPQVYTLPPSRDELTKNQVSLTCLVKGFYPSDIAVEWESNGQPENNYKTTPPVLDSDGSFFLYSKLTVDKSRWQQGNVFSCSVMHEALHNHYTQKSLSLSPG

SEQ ID NO: 12 - protein, 231 aa, Artificial Sequence
  hIgG1FcdeltaK-S Fc variant
EPKSSDKTHTCPPCPAPELLGGPSVFLFPPKPKDTLMISRTPEVTCVVVDVSHEDPEVKFNWYVDGVEVHNAKTKPREEQYNSTYRVVSVLTVLHQDWLNGKEYKCKVSNKALPAPIEKTISKAKGQPREPQVYTLPPSRDELTKNQVSLTCLVKGFYPSDIAVEWESNGQPENNYKTTPPVLDSDGSFFLYSKLTVDKSRWQQGNVFSCSVMHEALHNHYTQKSLSLSPG

SEQ ID NO: 13 - protein, 231 aa, Artificial Sequence; identical to SEQ ID NO: 12
  hIgG1deltaK-SS Fc variant

SEQ ID NO: 14 - protein, 231 aa, Artificial Sequence
  hIgG1FcdeltaK-SSS Fc variant
EPKSSDKTHTSPPSPAPELLGGPSVFLFPPKPKDTLMISRTPEVTCVVVDVSHEDPEVKFNWYVDGVEVHNAKTKPREEQYNSTYRVVSVLTVLHQDWLNGKEYKCKVSNKALPAPIEKTISKAKGQPREPQVYTLPPSRDELTKNQVSLTCLVKGFYPSDIAVEWESNGQPENNYKTTPPVLDSDGSFFLYSKLTVDKSRWQQGNVFSCSVMHEALHNHYTQKSLSLSPG

SEQ ID NO: 15 - protein, 215 aa, Artificial Sequence
  hIgG2FcdeltaK-deltaC Fc variant
APPVAGPSVFLFPPKPKDTLMISRTPEVTCVVVDVSHEDPEVQFNWYVDGVEVHNAKTKPREEQFNSTFRVVSVLTVVHQDWLNGKEYKCKVSNKGLPAPIEKTISKTKGQPREPQVYTLPPSREEMTKNQVSLTCLVKGFYPSDISVEWESNGQPENNYKTTPPMLDSDGSFFLYSKLTVDKSRWQQGNVFSCSVMHEALHNHYTQKSLSLSPG

SEQ ID NO: 16 - protein, 219 aa, Artificial Sequence
  hIgG2FcdeltaK-C Fc variant
PPCPAPPVAGPSVFLFPPKPKDTLMISRTPEVTCVVVDVSHEDPEVQFNWYVDGVEVHNAKTKPREEQFNSTFRVVSVLTVVHQDWLNGKEYKCKVSNKGLPAPIEKTISKTKGQPREPQVYTLPPSREEMTKNQVSLTCLVKGFYPSDISVEWESNGQPENNYKTTPPMLDSDGSFFLYSKLTVDKSRWQQGNVFSCSVMHEALHNHYTQKSLSLSPG

SEQ ID NO: 17 - protein, 222 aa, Artificial Sequence
  hIgG2FcdeltaK-CC Fc variant
VECPPCPAPPVAGPSVFLFPPKPKDTLMISRTPEVTCVVVDVSHEDPEVQFNWYVDGVEVHNAKTKPREEQFNSTFRVVSVLTVVHQDWLNGKEYKCKVSNKGLPAPIEKTISKTKGQPREPQVYTLPPSREEMTKNQVSLTCLVKGFYPSDISVEWESNGQPENNYKTTPPMLDSDGSFFLYSKLTVDKSRWQQGNVFSCSVMHEALHNHYTQKSLSLSPG

SEQ ID NO: 18 - protein, 228 aa, Artificial Sequence
  hIgG2Fc-CCCC Fc variant
ERKCCVECPPCPAPPVAGPSVFLFPPKPKDTLMISRTPEVTCVVVDVSHEDPEVQFNWYVDGVEVHNAKTKPREEQFNSTFRVVSVLTVVHQDWLNGKEYKCKVSNKGLPAPIEKTISKTKGQPREPQVYTLPPSREEMTKNQVSLTCLVKGFYPSDISVEWESNGQPENNYKTTPPMLDSDGSFFLYSKLTVDKSRWQQGNVFSCSVMHEALHNHYTQKSLSLSPGK

SEQ ID NO: 19 - protein, 227 aa, Artificial Sequence
  hIgG2FcdeltaK-SS Fc variant
ERKSSVECPPCPAPPVAGPSVFLFPPKPKDTLMISRTPEVTCVVVDVSHEDPEVQFNWYVDGVEVHNAKTKPREEQFNSTFRVVSVLTVVHQDWLNGKEYKCKVSNKGLPAPIEKTISKTKGQPREPQVYTLPPSREEMTKNQVSLTCLVKGFYPSDISVEWESNGQPENNYKTTPPMLDSDGSFFLYSKLTVDKSRWQQGNVFSCSVMHEALHNHYTQKSLSLSPG

SEQ ID NO: 20 - protein, 227 aa, Artificial Sequence
  hIgG2FcdeltaK-SSS Fc variant
ERKSSVESPPCPAPPVAGPSVFLFPPKPKDTLMISRTPEVTCVVVDVSHEDPEVQFNWYVDGVEVHNAKTKPREEQFNSTFRVVSVLTVVHQDWLNGKEYKCKVSNKGLPAPIEKTISKTKGQPREPQVYTLPPSREEMTKNQVSLTCLVKGFYPSDISVEWESNGQPENNYKTTPPMLDSDGSFFLYSKLTVDKSRWQQGNVFSCSVMHEALHNHYTQKSLSLSPG

SEQ ID NO: 21 - protein, 227 aa, Artificial Sequence
  hIgG2FcdeltaK-SSSS Fc variant
ERKSSVESPPSPAPPVAGPSVFLFPPKPKDTLMISRTPEVTCVVVDVSHEDPEVQFNWYVDGVEVHNAKTKPREEQFNSTFRVVSVLTVVHQDWLNGKEYKCKVSNKGLPAPIEKTISKTKGQPREPQVYTLPPSREEMTKNQVSLTCLVKGFYPSDISVEWESNGQPENNYKTTPPMLDSDGSFFLYSKLTVDKSRWQQGNVFSCSVMHEALHNHYTQKSLSLSPG

SEQ ID NO: 22 - protein, 216 aa, Artificial Sequence
  hIgG3FcdeltaK-deltaC Fc variant
APELLGGPSVFLFPPKPKDTLMISRTPEVTCVVVDVSHEDPEVQFKWYVDGVEVHNAKTKPREEQYNSTFRVVSVLTVLHQDWLNGKEYKCKVSNKALPAPIEKTISKTKGQPREPQVYTLPPSREEMTKNQVSLTCLVKGFYPSDIAVEWESSGQPENNYNTTPPMLDSDGSFFLYSKLTVDKSRWQQGNIFSCSVMHEALHNRFTQKSLSLSPG

SEQ ID NO: 23 - protein, 220 aa, Artificial Sequence
  hIgG3FcdeltaK-C Fc variant
PRCPAPELLGGPSVFLFPPKPKDTLMISRTPEVTCVVVDVSHEDPEVQFKWYVDGVEVHNAKTKPREEQYNSTFRVVSVLTVLHQDWLNGKEYKCKVSNKALPAPIEKTISKTKGQPREPQVYTLPPSREEMTKNQVSLTCLVKGFYPSDIAVEWESSGQPENNYNTTPPMLDSDGSFFLYSKLTVDKSRWQQGNIFSCSVMHEALHNRFTQKSLSLSPG

SEQ ID NO: 24 - protein, 226 aa, Artificial Sequence
  hIgG3FcdeltaK-CC Fc variant
DTPPPCPRCPAPELLGGPSVFLFPPKPKDTLMISRTPEVTCVVVDVSHEDPEVQFKWYVDGVEVHNAKTKPREEQYNSTFRVVSVLTVLHQDWLNGKEYKCKVSNKALPAPIEKTISKTKGQPREPQVYTLPPSREEMTKNQVSLTCLVKGFYPSDIAVEWESSGQPENNYNTTPPMLDSDGSFFLYSKLTVDKSRWQQGNIFSCSVMHEALHNRFTQKSLSLSPG

SEQ ID NO: 25 - protein, 231 aa, Artificial Sequence
  hIgG3FcdeltaK-S Fc variant
EPKSSDTPPPCPRCPAPELLGGPSVFLFPPKPKDTLMISRTPEVTCVVVDVSHEDPEVQFKWYVDGVEVHNAKTKPREEQYNSTFRVVSVLTVLHQDWLNGKEYKCKVSNKALPAPIEKTISKTKGQPREPQVYTLPPSREEMTKNQVSLTCLVKGFYPSDIAVEWESSGQPENNYNTTPPMLDSDGSFFLYSKLTVDKSRWQQGNIFSCSVMHEALHNRFTQKSLSLSPG

SEQ ID NO: 26 - protein, 231 aa, Artificial Sequence
  hIgG3FcdeltaK-SS Fc variant
EPKSSDTPPPSPRCPAPELLGGPSVFLFPPKPKDTLMISRTPEVTCVVVDVSHEDPEVQFKWYVDGVEVHNAKTKPREEQYNSTFRVVSVLTVLHQDWLNGKEYKCKVSNKALPAPIEKTISKTKGQPREPQVYTLPPSREEMTKNQVSLTCLVKGFYPSDIAVEWESSGQPENNYNTTPPMLDSDGSFFLYSKLTVDKSRWQQGNIFSCSVMHEALHNRFTQKSLSLSPG

SEQ ID NO: 27 - protein, 231 aa, Artificial Sequence
  hIgG3FcdeltaK-SSS Fc variant
EPKSSDTPPPSPRSPAPELLGGPSVFLFPPKPKDTLMISRTPEVTCVVVDVSHEDPEVQFKWYVDGVEVHNAKTKPREEQYNSTFRVVSVLTVLHQDWLNGKEYKCKVSNKALPAPIEKTISKTKGQPREPQVYTLPPSREEMTKNQVSLTCLVKGFYPSDIAVEWESSGQPENNYNTTPPMLDSDGSFFLYSKLTVDKSRWQQGNIFSCSVMHEALHNRFTQKSLSLSPG

SEQ ID NO: 28 - protein, 216 aa, Artificial Sequence
  hIgG4FcdeltaK-deltaC Fc variant
APEFLGGPSVFLFPPKPKDTLMISRTPEVTCVVVDVSQEDPEVQFNWYVDGVEVHNAKTKPREEQFNSTYRVVSVLTVLHQDWLNGKEYKCKVSNKGLPSSIEKTISKAKGQPREPQVYTLPPSQEEMTKNQVSLTCLVKGFYPSDIAVEWESNGQPENNYKTTPPVLDSDGSFFLYSRLTVDKSRWQEGNVFSCSVMHEALHNHYTQKSLSLSLG

SEQ ID NO: 29 - protein, 220 aa, Artificial Sequence
  hIgG4FcdeltaK-C Fc variant
PSCPAPEFLGGPSVFLFPPKPKDTLMISRTPEVTCVVVDVSQEDPEVQFNWYVDGVEVHNAKTKPREEQFNSTYRVVSVLTVLHQDWLNGKEYKCKVSNKGLPSSIEKTISKAKGQPREPQVYTLPPSQEEMTKNQVSLTCLVKGFYPSDIAVEWESNGQPENNYKTTPPVLDSDGSFFLYSRLTVDKSRWQEGNVFSCSVMHEALHNHYTQKSLSLSLG

SEQ ID NO: 30 - protein, 228 aa, Artificial Sequence
  hIgG4FcdeltaK-CC Fc variant
ESKYGPPCPSCPAPEFLGGPSVFLFPPKPKDTLMISRTPEVTCVVVDVSQEDPEVQFNWYVDGVEVHNAKTKPREEQFNSTYRVVSVLTVLHQDWLNGKEYKCKVSNKGLPSSIEKTISKAKGQPREPQVYTLPPSQEEMTKNQVSLTCLVKGFYPSDIAVEWESNGQPENNYKTTPPVLDSDGSFFLYSRLTVDKSRWQEGNVFSCSVMHEALHNHYTQKSLSLSLG

SEQ ID NO: 31 - protein, 228 aa, Artificial Sequence
  hIgG4FcdeltaK-CC-228P Fc variant
ESKYGPPCPPCPAPEFLGGPSVFLFPPKPKDTLMISRTPEVTCVVVDVSQEDPEVQFNWYVDGVEVHNAKTKPREEQFNSTYRVVSVLTVLHQDWLNGKEYKCKVSNKGLPSSIEKTISKAKGQPREPQVYTLPPSQEEMTKNQVSLTCLVKGFYPSDIAVEWESNGQPENNYKTTPPVLDSDGSFFLYSRLTVDKSRWQEGNVFSCSVMHEALHNHYTQKSLSLSLG

SEQ ID NO: 32 - protein, 228 aa, Artificial Sequence
  hIgG4FcdeltaK-CC-228P-409K Fc variant
ESKYGPPCPPCPAPEFLGGPSVFLFPPKPKDTLMISRTPEVTCVVVDVSQEDPEVQFNWYVDGVEVHNAKTKPREEQFNSTYRVVSVLTVLHQDWLNGKEYKCKVSNKGLPSSIEKTISKAKGQPREPQVYTLPPSQEEMTKNQVSLTCLVKGFYPSDIAVEWESNGQPENNYKTTPPVLDSDGSFFLYSKLTVDKSRWQEGNVFSCSVMHEALHNHYTQKSLSLSLG

SEQ ID NO: 33 - protein, 228 aa, Artificial Sequence
  hIgG4FcdeltaK-S Fc variant
ESKYGPPSPSCPAPEFLGGPSVFLFPPKPKDTLMISRTPEVTCVVVDVSQEDPEVQFNWYVDGVEVHNAKTKPREEQFNSTYRVVSVLTVLHQDWLNGKEYKCKVSNKGLPSSIEKTISKAKGQPREPQVYTLPPSQEEMTKNQVSLTCLVKGFYPSDIAVEWESNGQPENNYKTTPPVLDSDGSFFLYSRLTVDKSRWQEGNVFSCSVMHEALHNHYTQKSLSLSLG

SEQ ID NO: 34 - protein, 228 aa, Artificial Sequence
  hIgG4FcdeltaK-SS Fc variant
ESKYGPPSPSSPAPEFLGGPSVFLFPPKPKDTLMISRTPEVTCVVVDVSQEDPEVQFNWYVDGVEVHNAKTKPREEQFNSTYRVVSVLTVLHQDWLNGKEYKCKVSNKGLPSSIEKTISKAKGQPREPQVYTLPPSQEEMTKNQVSLTCLVKGFYPSDIAVEWESNGQPENNYKTTPPVLDSDGSFFLYSRLTVDKSRWQEGNVFSCSVMHEALHNHYTQKSLSLSLG

SEQ ID NO: 35 - protein, 101 aa, Artificial Sequence
  TbetaRII-ED structured domain
QLCKFCDVRFSTCDNQKSCMSNCSITSICEKPQEVCVAVWRKNDENITLETVCHDPKLPYHDFILEDAASPKCIMKEKKKPGETFFMCSCSSDECNDNIIF

SEQ ID NO: 36 - protein, 25 aa, Artificial Sequence
  TbetaRII-ED N-term unstructured region and natural linker
IPPHVQKSVNNDMIVTDNNGAVKFP

SEQ ID NO: 37 - protein, 50 aa, Artificial Sequence
  TbetaRIIb-ED N-term unstructured region and natural linker
IPPHVQKSDVEMEAQKDEIICPSCNRTAHPLRHINNDMIVTDNNGAVKFP

SEQ ID NO: 38 - protein, 50 aa, Artificial Sequence
  TbetaRIIb-ED Cys-mutated N-term unstructured region and natural linker
IPPHVQKSDVEMEAQKDEIIAPSANRTAHPLRHINNDMIVTDNNGAVKFP

SEQ ID NO: 39 - protein, 10 aa, Artificial Sequence
  TbetaRII-ED C-term unstructured region and natural linker
SEEYNTSNPD

SEQ ID NO: 40 - protein, 35 aa, Artificial Sequence
  TbetaRII-ED natural linker
SEEYNTSNPDIPPHVQKSVNNDMIVTDNNGAVKFP

SEQ ID NO: 41 - protein, 60 aa, Artificial Sequence
  TbetaRIIb-ED natural linker
SEEYNTSNPDIPPHVQKSDVEMEAQKDEIICPSCNRTAHPLRHINNDMIVTDNNGAVKFP

SEQ ID NO: 42 - protein, 60 aa, Artificial Sequence
  TbetaRIIb-ED Cys-mutated linker
SEEYNTSNPDIPPHVQKSDVEMEAQKDEIIAPSANRTAHPLRHINNDMIVTDNNGAVKFP

SEQ ID NO: 43 - protein, 136 aa, Artificial Sequence
  TbetaRII-ED monomer, also termed T2 or T2m
IPPHVQKSVNNDMIVTDNNGAVKFPQLCKFCDVRFSTCDNQKSCMSNCSITSICEKPQEVCVAVWRKNDENITLETVCHDPKLPYHDFILEDAASPKCIMKEKKKPGETFFMCSCSSDECNDNIIFSEEYNTSNPD

SEQ ID NO: 44 - protein, 161 aa, Artificial Sequence
  TbetabRIIb-ED monomer, also termed T2b
IPPHVQKSDVEMEAQKDEIICPSCNRTAHPLRHINNDMIVTDNNGAVKFPQLCKFCDVRFSTCDNQKSCMSNCSITSICEKPQEVCVAVWRKNDENITLETVCHDPKLPYHDFILEDAASPKCIMKEKKKPGETFFMCSCSSDECNDNIIFSEEYNTSNPD

SEQ ID NO: 45 - protein, 161 aa, Artificial Sequence
  TbetaRIIb-ED monomer Cys-mutated in the linker region, also termed T2bAA
IPPHVQKSDVEMEAQKDEIIAPSANRTAHPLRHINNDMIVTDNNGAVKFPQLCKFCDVRFSTCDNQKSCMSNCSITSICEKPQEVCVAVWRKNDENITLETVCHDPKLPYHDFILEDAASPKCIMKEKKKPGETFFMCSCSSDECNDNIIFSEEYNTSNPD

SEQ ID NO: 46 - protein, 272 aa, Artificial Sequence
  TbetaRII-ED dimer, also termed T2-T2 or T22d35
IPPHVQKSVNNDMIVTDNNGAVKFPQLCKFCDVRFSTCDNQKSCMSNCSITSICEKPQEVCVAVWRKNDENITLETVCHDPKLPYHDFILEDAASPKCIMKEKKKPGETFFMCSCSSDECNDNIIFSEEYNTSNPDIPPHVQKSVNNDMIVTDNNGAVKFPQLCKFCDVRFSTCDNQKSCMSNCSITSICEKPQEVCVAVWRKNDENITLETVCHDPKLPYHDFILEDAASPKCIMKEKKKPGETFFMCSCSSDECNDNIIFSEEYNTSNPD

SEQ ID NO: 47 - protein, 322 aa, Artificial Sequence
  TbetaRIIb-ED dimer, also termed T2-T2b
IPPHVQKSDVEMEAQKDEIICPSCNRTAHPLRHINNDMIVTDNNGAVKFPQLCKFCDVRFSTCDNQKSCMSNCSITSICEKPQEVCVAVWRKNDENITLETVCHDPKLPYHDFILEDAASPKCIMKEKKKPGETFFMCSCSSDECNDNIIFSEEYNTSNPDIPPHVQKSDVEMEAQKDEIICPSCNRTAHPLRHINNDMIVTDNNGAVKFPQLCKFCDVRFSTCDNQKSCMSNCSITSICEKPQEVCVAVWRKNDENITLETVCHDPKLPYHDFILEDAASPKCIMKEKKKPGETFFMCSCSSDECNDNIIFSEEYNTSNPD

SEQ ID NO: 48 - protein, 322 aa, Artificial Sequence
  TbetaRIIb-ED dimer Cys-mutated in the linker region, also termed T2-T2bAA
IPPHVQKSDVEMEAQKDEIICPSCNRTAHPLRHINNDMIVTDNNGAVKFPQLCKFCDVRFSTCDNQKSCMSNCSITSICEKPQEVCVAVWRKNDENITLETVCHDPKLPYHDFILEDAASPKCIMKEKKKPGETFFMCSCSSDECNDNIIFSEEYNTSNPDIPPHVQKSDVEMEAQKDEIIAPSANRTAHPLRHINNDMIVTDNNGAVKFPQLCKFCDVRFSTCDNQKSCMSNCSITSICEKPQEVCVAVWRKNDENITLETVCHDPKLPYHDFILEDAASPKCIMKEKKKPGETFFMCSCSSDECNDNIIFSEEYNTSNPD

SEQ ID NO: 49 - protein, 408 aa, Artificial Sequence
  TbetaRII-ED trimer, also termed T2-T2-T2
IPPHVQKSVNNDMIVTDNNGAVKFPQLCKFCDVRFSTCDNQKSCMSNCSITSICEKPQEVCVAVWRKNDENITLETVCHDPKLPYHDFILEDAASPKCIMKEKKKPGETFFMCSCSSDECNDNIIFSEEYNTSNPDIPPHVQKSVNNDMIVTDNNGAVKFPQLCKFCDVRFSTCDNQKSCMSNCSITSICEKPQEVCVAVWRKNDENITLETVCHDPKLPYHDFILEDAASPKCIMKEKKKPGETFFMCSCSSDECNDNIIFSEEYNTSNPDIPPHVQKSVNNDMIVTDNNGAVKFPQLCKFCDVRFSTCDNQKSCMSNCSITSICEKPQEVCVAVWRKNDENITLETVCHDPKLPYHDFILEDAASPKCIMKEKKKPGETFFMCSCSSDECNDNIIFSEEYNTSNPD

SEQ ID NO: 50 - protein, 458 aa, Artificial Sequence
  TbetaRIIb-ED trimer, also termed T2-T2b-T2b
IPPHVQKSVNNDMIVTDNNGAVKFPQLCKFCDVRFSTCDNQKSCMSNCSITSICEKPQEVCVAVWRKNDENITLETVCHDPKLPYHDFILEDAASPKCIMKEKKKPGETFFMCSCSSDECNDNIIFSEEYNTSNPDIPPHVQKSDVEMEAQKDEIICPSCNRTAHPLRHINNDMIVTDNNGAVKFPQLCKFCDVRFSTCDNQKSCMSNCSITSICEKPQEVCVAVWRKNDENITLETVCHDPKLPYHDFILEDAASPKCIMKEKKKPGETFFMCSCSSDECNDNIIFSEEYNTSNPDIPPHVQKSDVEMEAQKDEIICPSCNRTAHPLRHINNDMIVTDNNGAVKFPQLCKFCDVRFSTCDNQKSCMSNCSITSICEKPQEVCVAVWRKNDENITLETVCHDPKLPYHDFILEDAASPKCIMKEKKKPGETFFMCSCSSDECNDNIIFSEEYNTSNPD

SEQ ID NO: 51 - protein, 458 aa, Artificial Sequence
  TbetaRIIb-ED trimer Cys-mutated in the linker regions, also termed T2-T2bAA-T2bAA
IPPHVQKSVNNDMIVTDNNGAVKFPQLCKFCDVRFSTCDNQKSCMSNCSITSICEKPQEVCVAVWRKNDENITLETVCHDPKLPYHDFILEDAASPKCIMKEKKKPGETFFMCSCSSDECNDNIIFSEEYNTSNPDIPPHVQKSDVEMEAQKDEIIAPSANRTAHPLRHINNDMIVTDNNGAVKFPQLCKFCDVRFSTCDNQKSCMSNCSITSICEKPQEVCVAVWRKNDENITLETVCHDPKLPYHDFILEDAASPKCIMKEKKKPGETFFMCSCSSDECNDNIIFSEEYNTSNPDIPPHVQKSDVEMEAQKDEIIAPSANRTAHPLRHINNDMIVTDNNGAVKFPQLCKFCDVRFSTCDNQKSCMSNCSITSICEKPQEVCVAVWRKNDENITLETVCHDPKLPYHDFILEDAASPKCIMKEKKKPGETFFMCSCSSDECNDNIIFSEEYNTSNPD

SEQ ID NO: 52 - protein, 79 aa, Artificial Sequence
  TbetaRI-ED structured domain
ALQCFCHLCTKDNFTCVTDGLCFVSVTETTDKVIHNSMCIAEIDLIPRDRPFVCAPSSKTGSVTTTYCCNQDHCNKIEL

SEQ ID NO: 53 - protein, 8 aa, Artificial Sequence
  TbetaRI-ED N-term unstructured region and natural linker
AALLPGAT

SEQ ID NO: 54 - protein, 14 aa, Artificial Sequence
  TbetaRI-ED C-term unstructured region and natural linker
PTTVKSSPGLGPVE

SEQ ID NO: 55 - protein, 22 aa, Artificial Sequence
  TbetaRI-ED natural linker
PTTVKSSPGLGPVEAALLPGAT

SEQ ID NO: 56 - protein, 101 aa, Artificial Sequence
  TbetaRI-ED monomer, also termed T1 or T1m
AALLPGATALQCFCHLCTKDNFTCVTDGLCFVSVTETTDKVIHNSMCIAEIDLIPRDRPFVCAPSSKTGSVTTTYCCNQDHCNKIELPTTVKSSPGLGPVE

SEQ ID NO: 57 - protein, 202 aa, Artificial Sequence
  TbetaRI-ED dimer, also termed T1-T1
AALLPGATALQCFCHLCTKDNFTCVTDGLCFVSVTETTDKVIHNSMCIAEIDLIPRDRPFVCAPSSKTGSVTTTYCCNQDHCNKIELPTTVKSSPGLGPVEAALLPGATALQCFCHLCTKDNFTCVTDGLCFVSVTETTDKVIHNSMCIAEIDLIPRDRPFVCAPSSKTGSVTTTYCCNQDHCNKIELPTTVKSSPGLGPVE

SEQ ID NO: 58 - protein, 39 aa, Artificial Sequence
  TbetaRI-TbetaRII-ED natural linker
PTTVKSSPGLGPVEIPPHVQKSVNNDMIVTDNNGAVKFP

SEQ ID NO: 59 - protein, 64 aa, Artificial Sequence
  TbetaRI-TbetaRIIb-ED natural linker
PTTVKSSPGLGPVEIPPHVQKSDVEMEAQKDEIICPSCNRTAHPLRHINNDMIVTDNNGAVKFP

SEQ ID NO: 60 - protein, 18 aa, Artificial Sequence
  TbetaRII-TbetaRI-ED natural linker
SEEYNTSNPDAALLPGAT

SEQ ID NO: 61 - protein, 237 aa, Artificial Sequence
  TbetaRI-TbetaRII-ED dimer T1-T2
AALLPGATALQCFCHLCTKDNFTCVTDGLCFVSVTETTDKVIHNSMCIAEIDLIPRDRPFVCAPSSKTGSVTTTYCCNQDHCNKIELPTTVKSSPGLGPVEIPPHVQKSVNNDMIVTDNNGAVKFPQLCKFCDVRFSTCDNQKSCMSNCSITSICEKPQEVCVAVWRKNDENITLETVCHDPKLPYHDFILEDAASPKCIMKEKKKPGETFFMCSCSSDECNDNIIFSEEYNTSNPD

SEQ ID NO: 62 - protein, 262 aa, Artificial Sequence
  TbetaRI-TbetaRII-ED dimer T1-T2b
AALLPGATALQCFCHLCTKDNFTCVTDGLCFVSVTETTDKVIHNSMCIAEIDLIPRDRPFVCAPSSKTGSVTTTYCCNQDHCNKIELPTTVKSSPGLGPVEIPPHVQKSDVEMEAQKDEIICPSCNRTAHPLRHINNDMIVTDNNGAVKFPQLCKFCDVRFSTCDNQKSCMSNCSITSICEKPQEVCVAVWRKNDENITLETVCHDPKLPYHDFILEDAASPKCIMKEKKKPGETFFMCSCSSDECNDNIIFSEEYNTSNPD

SEQ ID NO: 63 - protein, 237 aa, Artificial Sequence
  TbetaRI-TbetaRII-ED dimer T2-T1
IPPHVQKSVNNDMIVTDNNGAVKFPQLCKFCDVRFSTCDNQKSCMSNCSITSICEKPQEVCVAVWRKNDENITLETVCHDPKLPYHDFILEDAASPKCIMKEKKKPGETFFMCSCSSDECNDNIIFSEEYNTSNPDAALLPGATALQCFCHLCTKDNFTCVTDGLCFVSVTETTDKVIHNSMCIAEIDLIPRDRPFVCAPSSKTGSVTTTYCCNQDHCNKIELPTTVKSSPGLGPVE

SEQ ID NO: 64 - protein, 373 aa, Artificial Sequence
  TbetaRI-TbetaRII-ED trimer T1-T2-T2
AALLPGATALQCFCHLCTKDNFTCVTDGLCFVSVTETTDKVIHNSMCIAEIDLIPRDRPFVCAPSSKTGSVTTTYCCNQDHCNKIELPTTVKSSPGLGPVEIPPHVQKSVNNDMIVTDNNGAVKFPQLCKFCDVRFSTCDNQKSCMSNCSITSICEKPQEVCVAVWRKNDENITLETVCHDPKLPYHDFILEDAASPKCIMKEKKKPGETFFMCSCSSDECNDNIIFSEEYNTSNPDIPPHVQKSVNNDMIVTDNNGAVKFPQLCKFCDVRFSTCDNQKSCMSNCSITSICEKPQEVCVAVWRKNDENITLETVCHDPKLPYHDFILEDAASPKCIMKEKKKPGETFFMCSCSSDECNDNIIFSEEYNTSNPD

SEQ ID NO: 65 - protein, 398 aa, Artificial Sequence
  TbetaRI-TbetaRII-ED trimer T1-T2-T2b
AALLPGATALQCFCHLCTKDNFTCVTDGLCFVSVTETTDKVIHNSMCIAEIDLIPRDRPFVCAPSSKTGSVTTTYCCNQDHCNKIELPTTVKSSPGLGPVEIPPHVQKSVNNDMIVTDNNGAVKFPQLCKFCDVRFSTCDNQKSCMSNCSITSICEKPQEVCVAVWRKNDENITLETVCHDPKLPYHDFILEDAASPKCIMKEKKKPGETFFMCSCSSDECNDNIIFSEEYNTSNPDIPPHVQKSDVEMEAQKDEIICPSCNRTAHPLRHINNDMIVTDNNGAVKFPQLCKFCDVRFSTCDNQKSCMSNCSITSICEKPQEVCVAVWRKNDENITLETVCHDPKLPYHDFILEDAASPKCIMKEKKKPGETFFMCSCSSDECNDNIIFSEEYNTSNPD

SEQ ID NO: 66 - protein, 423 aa, Artificial Sequence
  TbetaRI-TbetaRII-ED trimer T1-T2-T2bAA
AALLPGATALQCFCHLCTKDNFTCVTDGLCFVSVTETTDKVIHNSMCIAEIDLIPRDRPFVCAPSSKTGSVTTTYCCNQDHCNKIELPTTVKSSPGLGPVEIPPHVQKSDVEMEAQKDEIICPSCNRTAHPLRHINNDMIVTDNNGAVKFPQLCKFCDVRFSTCDNQKSCMSNCSITSICEKPQEVCVAVWRKNDENITLETVCHDPKLPYHDFILEDAASPKCIMKEKKKPGETFFMCSCSSDECNDNIIFSEEYNTSNPDIPPHVQKSDVEMEAQKDEIIAPSANRTAHPLRHINNDMIVTDNNGAVKFPQLCKFCDVRFSTCDNQKSCMSNCSITSICEKPQEVCVAVWRKNDENITLETVCHDPKLPYHDFILEDAASPKCIMKEKKKPGETFFMCSCSSDECNDNIIFSEEYNTSNPD

SEQ ID NO: 67 - protein, 373 aa, Artificial Sequence
  TbetaRI-TbetaRII-ED trimer T2-T2-T1
IPPHVQKSVNNDMIVTDNNGAVKFPQLCKFCDVRFSTCDNQKSCMSNCSITSICEKPQEVCVAVWRKNDENITLETVCHDPKLPYHDFILEDAASPKCIMKEKKKPGETFFMCSCSSDECNDNIIFSEEYNTSNPDIPPHVQKSVNNDMIVTDNNGAVKFPQLCKFCDVRFSTCDNQKSCMSNCSITSICEKPQEVCVAVWRKNDENITLETVCHDPKLPYHDFILEDAASPKCIMKEKKKPGETFFMCSCSSDECNDNIIFSEEYNTSNPDAALLPGATALQCFCHLCTKDNFTCVTDGLCFVSVTETTDKVIHNSMCIAEIDLIPRDRPFVCAPSSKTGSVTTTYCCNQDHCNKIELPTTVKSSPGLGPVE

SEQ ID NO: 68 - protein, 398 aa, Artificial Sequence
  TbetaRI-TbetaRII-ED trimer T2-T2bAA-T1
IPPHVQKSVNNDMIVTDNNGAVKFPQLCKFCDVRFSTCDNQKSCMSNCSITSICEKPQEVCVAVWRKNDENITLETVCHDPKLPYHDFILEDAASPKCIMKEKKKPGETFFMCSCSSDECNDNIIFSEEYNTSNPDIPPHVQKSDVEMEAQKDEIIAPSANRTAHPLRHINNDMIVTDNNGAVKFPQLCKFCDVRFSTCDNQKSCMSNCSITSICEKPQEVCVAVWRKNDENITLETVCHDPKLPYHDFILEDAASPKCIMKEKKKPGETFFMCSCSSDECNDNIIFSEEYNTSNPDAALLPGATALQCFCHLCTKDNFTCVTDGLCFVSVTETTDKVIHNSMCIAEIDLIPRDRPFVCAPSSKTGSVTTTYCCNQDHCNKIELPTTVKSSPGLGPVE

SEQ ID NO: 69 - protein, 85 aa, Artificial Sequence
  BMPRIa-ED structured domain
TLPFLKCYCSGHCPDDAINNTCITNGHCFAIIEEDDQGETTLASGCMKYEGSDFQCKDSPKAQLRRTIECCRTNLCNQYLQPTLP

SEQ ID NO: 70 - protein, 31 aa, Artificial Sequence
  BMPRIa-ED N-term unstructured region and natural linker
QNLDSMLHGTGMKSDSDQKKSENGVTLAPED

SEQ ID NO: 71 - protein, 13 aa, Artificial Sequence
  BMPRIa-ED C-term unstructured region and natural linker
PVVIGPFFDGSIR

SEQ ID NO: 72 - protein, 44 aa, Artificial Sequence
  BMPRIa-ED natural linker
PVVIGPFFDGSIRQNLDSMLHGTGMKSDSDQKKSENGVTLAPED

SEQ ID NO: 73 - protein, 129 aa, Artificial Sequence
  BMPRIa-ED monomer
QNLDSMLHGTGMKSDSDQKKSENGVTLAPEDTLPFLKCYCSGHCPDDAINNTCITNGHCFAIIEEDDQGETTLASGCMKYEGSDFQCKDSPKAQLRRTIECCRTNLCNQYLQPTLPPVVIGPFFDGSIR

SEQ ID NO: 74 - protein, 258 aa, Artificial Sequence
  BMPRIa-ED dimer
QNLDSMLHGTGMKSDSDQKKSENGVTLAPEDTLPFLKCYCSGHCPDDAINNTCITNGHCFAIIEEDDQGETTLASGCMKYEGSDFQCKDSPKAQLRRTIECCRTNLCNQYLQPTLPPVVIGPFFDGSIRQNLDSMLHGTGMKSDSDQKKSENGVTLAPEDTLPFLKCYCSGHCPDDAINNTCITNGHCFAIIEEDDQGETTLASGCMKYEGSDFQCKDSPKAQLRRTIECCRTNLCNQYLQPTLPPVVIGPFFDGSIR

SEQ ID NO: 75 - protein, 92 aa, Artificial Sequence
  ActRIIa-ED structured domain
TQECLFFNANWEKDRTNQTGVEPCYGDKDKRRHCFATWKNISGSIEIVKQGCWLDDINCYDRTDCVEKKDSPEVYFCCCEGNMCNEKFSYFP

SEQ ID NO: 76 - protein, 7 aa, Artificial Sequence
  ActRIIa-ED N-term unstructured region and natural linker
AILGRSE

SEQ ID NO: 77 - protein, 21 aa, Artificial Sequence
  ActRIIa-ED C-term unstructured region and natural linker
EMEVTQPTSNPVTPKPPYYNI

SEQ ID NO: 78 - protein, 28 aa, Artificial Sequence
  ActRIIa-ED natural linker
EMEVTQPTSNPVTPKPPYYNIAILGRSE

SEQ ID NO: 79 - protein, 120 aa, Artificial Sequence
  ActRIIa-ED monomer
AILGRSETQECLFFNANWEKDRTNQTGVEPCYGDKDKRRHCFATWKNISGSIEIVKQGCWLDDINCYDRTDCVEKKDSPEVYFCCCEGNMCNEKFSYFPEMEVTQPTSNPVTPKPPYYNI

SEQ ID NO: 80 - protein, 240 aa, Artificial Sequence
  ActRIIa-ED dimer
AILGRSETQECLFFNANWEKDRTNQTGVEPCYGDKDKRRHCFATWKNISGSIEIVKQGCWLDDINCYDRTDCVEKKDSPEVYFCCCEGNMCNEKFSYFPEMEVTQPTSNPVTPKPPYYNIAILGRSETQECLFFNANWEKDRTNQTGVEPCYGDKDKRRHCFATWKNISGSIEIVKQGCWLDDINCYDRTDCVEKKDSPEVYFCCCEGNMCNEKFSYFPEMEVTQPTSNPVTPKPPYYNI

SEQ ID NO: 81 - protein, 91 aa, Artificial Sequence
  ActRIIb-ED structured domain
RECIYYNANWELERTNQSGLERCEGEQDKRLHCYASWRNSSGTIELVKKGCWLDDFNCYDRQECVATEENPQVYFCCCEGNFCNERFTHLP

SEQ ID NO: 82 - protein, 8 aa, Artificial Sequence
  ActRIIb-ED N-term unstructured region and natural linker
SGRGEAET

SEQ ID NO: 83 - protein, 17 aa, Artificial Sequence
  ActRIIb-ED C-term unstructured region and natural linker
EAGGPEVTYEPPPTAPT

SEQ ID NO: 84 - protein, 25 aa, Artificial Sequence
  ActRIIb-ED natural linker
EAGGPEVTYEPPPTAPTSGRGEAET

SEQ ID NO: 85 - protein, 116 aa, Artificial Sequence
  ActRIIb-ED monomer
SGRGEAETRECIYYNANWELERTNQSGLERCEGEQDKRLHCYASWRNSSGTIELVKKGCWLDDFNCYDRQECVATEENPQVYFCCCEGNFCNERFTHLPEAGGPEVTYEPPPTAPT

SEQ ID NO: 86 - protein, 232 aa, Artificial Sequence
  ActRIIb-ED dimer
SGRGEAETRECIYYNANWELERTNQSGLERCEGEQDKRLHCYASWRNSSGTIELVKKGCWLDDFNCYDRQECVATEENPQVYFCCCEGNFCNERFTHLPEAGGPEVTYEPPPTAPTSGRGEAETRECIYYNANWELERTNQSGLERCEGEQDKRLHCYASWRNSSGTIELVKKGCWLDDFNCYDRQECVATEENPQVYFCCCEGNFCNERFTHLPEAGGPEVTYEPPPTAPT

SEQ ID NO: 87 - protein, 52 aa, Artificial Sequence
  ActRIIa-BMPRIa-ED natural linker
EMEVTQPTSNPVTPKPPYYNIQNLDSMLHGTGMKSDSDQKKSENGVTLAPED

SEQ ID NO: 88 - protein, 249 aa, Artificial Sequence
  ActRIIa-BMPRIa-ED dimer
AILGRSETQECLFFNANWEKDRTNQTGVEPCYGDKDKRRHCFATWKNISGSIEIVKQGCWLDDINCYDRTDCVEKKDSPEVYFCCCEGNMCNEKFSYFPEMEVTQPTSNPVTPKPPYYNIQNLDSMLHGTGMKSDSDQKKSENGVTLAPEDTLPFLKCYCSGHCPDDAINNTCITNGHCFAIIEEDDQGETTLASGCMKYEGSDFQCKDSPKAQLRRTIECCRTNLCNQYLQPTLPPVVIGPFFDGSIR

SEQ ID NO: 89 - protein, 19 aa, Artificial Sequence
  Signal peptide
MDWTWRILFLVAAATGTHA

SEQ ID NO: 90 - protein, 20 aa, Artificial Sequence
  Signal peptide
MVLQTQVFISLLLWISGAYG

SEQ ID NO: 91 - protein, 352 aa, Artificial Sequence
  hIgG1FcdeltaK-deltaC-T2m fusion
APELLGGPSVFLFPPKPKDTLMISRTPEVTCVVVDVSHEDPEVKFNWYVDGVEVHNAKTKPREEQYNSTYRVVSVLTVLHQDWLNGKEYKCKVSNKALPAPIEKTISKAKGQPREPQVYTLPPSRDELTKNQVSLTCLVKGFYPSDIAVEWESNGQPENNYKTTPPVLDSDGSFFLYSKLTVDKSRWQQGNVFSCSVMHEALHNHYTQKSLSLSPGIPPHVQKSVNNDMIVTDNNGAVKFPQLCKFCDVRFSTCDNQKSCMSNCSITSICEKPQEVCVAVWRKNDENITLETVCHDPKLPYHDFILEDAASPKCIMKEKKKPGETFFMCSCSSDECNDNIIFSEEYNTSNPD

SEQ ID NO: 92 - protein, 356 aa, Artificial Sequence
  hIgG1FcdeltaK-C-T2m fusion
PPCPAPELLGGPSVFLFPPKPKDTLMISRTPEVTCVVVDVSHEDPEVKFNWYVDGVEVHNAKTKPREEQYNSTYRVVSVLTVLHQDWLNGKEYKCKVSNKALPAPIEKTISKAKGQPREPQVYTLPPSRDELTKNQVSLTCLVKGFYPSDIAVEWESNGQPENNYKTTPPVLDSDGSFFLYSKLTVDKSRWQQGNVFSCSVMHEALHNHYTQKSLSLSPGIPPHVQKSVNNDMIVTDNNGAVKFPQLCKFCDVRFSTCDNQKSCMSNCSITSICEKPQEVCVAVWRKNDENITLETVCHDPKLPYHDFILEDAASPKCIMKEKKKPGETFFMCSCSSDECNDNIIFSEEYNTSNPD

SEQ ID NO: 93 - protein, 362 aa, Artificial Sequence
  hIgG1FcdeltaK-CC-T2m fusion
DKTHTCPPCPAPELLGGPSVFLFPPKPKDTLMISRTPEVTCVVVDVSHEDPEVKFNWYVDGVEVHNAKTKPREEQYNSTYRVVSVLTVLHQDWLNGKEYKCKVSNKALPAPIEKTISKAKGQPREPQVYTLPPSRDELTKNQVSLTCLVKGFYPSDIAVEWESNGQPENNYKTTPPVLDSDGSFFLYSKLTVDKSRWQQGNVFSCSVMHEALHNHYTQKSLSLSPGIPPHVQKSVNNDMIVTDNNGAVKFPQLCKFCDVRFSTCDNQKSCMSNCSITSICEKPQEVCVAVWRKNDENITLETVCHDPKLPYHDFILEDAASPKCIMKEKKKPGETFFMCSCSSDECNDNIIFSEEYNTSNPD

SEQ ID NO: 94 - protein, 351 aa, Artificial Sequence
  hIgG2FcdeltaK-deltaC-T2m fusion
APPVAGPSVFLFPPKPKDTLMISRTPEVTCVVVDVSHEDPEVQFNWYVDGVEVHNAKTKPREEQFNSTFRVVSVLTVVHQDWLNGKEYKCKVSNKGLPAPIEKTISKTKGQPREPQVYTLPPSREEMTKNQVSLTCLVKGFYPSDISVEWESNGQPENNYKTTPPMLDSDGSFFLYSKLTVDKSRWQQGNVFSCSVMHEALHNHYTQKSLSLSPGIPPHVQKSVNNDMIVTDNNGAVKFPQLCKFCDVRFSTCDNQKSCMSNCSITSICEKPQEVCVAVWRKNDENITLETVCHDPKLPYHDFILEDAASPKCIMKEKKKPGETFFMCSCSSDECNDNIIFSEEYNTSNPD

SEQ ID NO: 95 - protein, 355 aa, Artificial Sequence
  hIgG2FcdeltaK-C-T2m fusion
PPCPAPPVAGPSVFLFPPKPKDTLMISRTPEVTCVVVDVSHEDPEVQFNWYVDGVEVHNAKTKPREEQFNSTFRVVSVLTVVHQDWLNGKEYKCKVSNKGLPAPIEKTISKTKGQPREPQVYTLPPSREEMTKNQVSLTCLVKGFYPSDISVEWESNGQPENNYKTTPPMLDSDGSFFLYSKLTVDKSRWQQGNVFSCSVMHEALHNHYTQKSLSLSPGIPPHVQKSVNNDMIVTDNNGAVKFPQLCKFCDVRFSTCDNQKSCMSNCSITSICEKPQEVCVAVWRKNDENITLETVCHDPKLPYHDFILEDAASPKCIMKEKKKPGETFFMCSCSSDECNDNIIFSEEYNTSNPD

SEQ ID NO: 96 - protein, 351 aa, Artificial Sequence; identical to SEQ ID NO: 94
  hIgG2FcdeltaK-CC-T2m fusion

SEQ ID NO: 97 - protein, 383 aa, Artificial Sequence
  hIgG2Fc-CCCC-T2 fusion, also termed Fc-T2m
MDWTWRILFLVAAATGTHAERKCCVECPPCPAPPVAGPSVFLFPPKPKDTLMISRTPEVTCVVVDVSHEDPEVQFNWYVDGVEVHNAKTKPREEQFNSTFRVVSVLTVVHQDWLNGKEYKCKVSNKGLPAPIEKTISKTKGQPREPQVYTLPPSREEMTKNQVSLTCLVKGFYPSDISVEWESNGQPENNYKTTPPMLDSDGSFFLYSKLTVDKSRWQQGNVFSCSVMHEALHNHYTQKSLSLSPGKIPPHVQKSVNNDMIVTDNNGAVKFPQLCKFCDVRFSTCDNQKSCMSNCSITSICEKPQEVCVAVWRKNDENITLETVCHDPKLPYHDFILEDAASPKCIMKEKKKPGETFFMCSCSSDECNDNIIFSEEYNTSNPD

SEQ ID NO: 98 - protein, 364 aa, Artificial Sequence
  hIgG4Fc K-CC-228P-T2m fusion
ESKYGPPCPPCPAPEFLGGPSVFLFPPKPKDTLMISRTPEVTCVVVDVSQEDPEVQFNWYVDGVEVHNAKTKPREEQFNSTYRVVSVLTVLHQDWLNGKEYKCKVSNKGLPSSIEKTISKAKGQPREPQVYTLPPSQEEMTKNQVSLTCLVKGFYPSDIAVEWESNGQPENNYKTTPPVLDSDGSFFLYSRLTVDKSRWQEGNVFSCSVMHEALHNHYTQKSLSLSLGIPPHVQKSVNNDMIVTDNNGAVKFPQLCKFCDVRFSTCDNQKSCMSNCSITSICEKPQEVCVAVWRKNDENITLETVCHDPKLPYHDFILEDAASPKCIMKEKKKPGETFFMCSCSSDECNDNIIFSEEYNTSNPD

SEQ ID NO: 99 - protein, 364 aa, Artificial Sequence
  hIgG4FcdeltaK-CC-228P-409K-T2m fusion
ESKYGPPCPPCPAPEFLGGPSVFLFPPKPKDTLMISRTPEVTCVVVDVSQEDPEVQFNWYVDGVEVHNAKTKPREEQFNSTYRVVSVLTVLHQDWLNGKEYKCKVSNKGLPSSIEKTISKAKGQPREPQVYTLPPSQEEMTKNQVSLTCLVKGFYPSDIAVEWESNGQPENNYKTTPPVLDSDGSFFLYSKLTVDKSRWQEGNVFSCSVMHEALHNHYTQKSLSLSLGIPPHVQKSVNNDMIVTDNNGAVKFPQLCKFCDVRFSTCDNQKSCMSNCSITSICEKPQEVCVAVWRKNDENITLETVCHDPKLPYHDFILEDAASPKCIMKEKKKPGETFFMCSCSSDECNDNIIFSEEYNTSNPD

SEQ ID NO: 100 - protein, 492 aa, Artificial Sequence
  hIgG1FcdeltaK-C-T22d35 fusion
PPCPAPELLGGPSVFLFPPKPKDTLMISRTPEVTCVVVDVSHEDPEVKFNWYVDGVEVHNAKTKPREEQYNSTYRVVSVLTVLHQDWLNGKEYKCKVSNKALPAPIEKTISKAKGQPREPQVYTLPPSRDELTKNQVSLTCLVKGFYPSDIAVEWESNGQPENNYKTTPPVLDSDGSFFLYSKLTVDKSRWQQGNVFSCSVMHEALHNHYTQKSLSLSPGIPPHVQKSVNNDMIVTDNNGAVKFPQLCKFCDVRFSTCDNQKSCMSNCSITSICEKPQEVCVAVWRKNDENITLETVCHDPKLPYHDFILEDAASPKCIMKEKKKPGETFFMCSCSSDECNDNIIFSEEYNTSNPDIPPHVQKSVNNDMIVTDNNGAVKFPQLCKFCDVRFSTCDNQKSCMSNCSITSICEKPQEVCVAVWRKNDENITLETVCHDPKLPYHDFILEDAASPKCIMKEKKKPGETFFMCSCSSDECNDNIIFSEEYNTSNPD

SEQ ID NO: 101 - protein, 498 aa, Artificial Sequence
  hIgG1FcdeltaK-CC-T22d35 fusion
DKTHTCPPCPAPELLGGPSVFLFPPKPKDTLMISRTPEVTCVVVDVSHEDPEVKFNWYVDGVEVHNAKTKPREEQYNSTYRVVSVLTVLHQDWLNGKEYKCKVSNKALPAPIEKTISKAKGQPREPQVYTLPPSRDELTKNQVSLTCLVKGFYPSDIAVEWESNGQPENNYKTTPPVLDSDGSFFLYSKLTVDKSRWQQGNVFSCSVMHEALHNHYTQKSLSLSPGIPPHVQKSVNNDMIVTDNNGAVKFPQLCKFCDVRFSTCDNQKSCMSNCSITSICEKPQEVCVAVWRKNDENITLETVCHDPKLPYHDFILEDAASPKCIMKEKKKPGETFFMCSCSSDECNDNIIFSEEYNTSNPDIPPHVQKSVNNDMIVTDNNGAVKFPQLCKFCDVRFSTCDNQKSCMSNCSITSICEKPQEVCVAVWRKNDENITLETVCHDPKLPYHDFILEDAASPKCIMKEKKKPGETFFMCSCSSDECNDNIIFSEEYNTSNPD

SEQ ID NO: 102 - protein, 494 aa, Artificial Sequence
  hIgG2FcdeltaK-CC-T22d35 fusion
VECPPCPAPPVAGPSVFLFPPKPKDTLMISRTPEVTCVVVDVSHEDPEVQFNWYVDGVEVHNAKTKPREEQFNSTFRVVSVLTVVHQDWLNGKEYKCKVSNKGLPAPIEKTISKTKGQPREPQVYTLPPSREEMTKNQVSLTCLVKGFYPSDISVEWESNGQPENNYKTTPPMLDSDGSFFLYSKLTVDKSRWQQGNVFSCSVMHEALHNHYTQKSLSLSPGIPPHVQKSVNNDMIVTDNNGAVKFPQLCKFCDVRFSTCDNQKSCMSNCSITSICEKPQEVCVAVWRKNDENITLETVCHDPKLPYHDFILEDAASPKCIMKEKKKPGETFFMCSCSSDECNDNIIFSEEYNTSNPDIPPHVQKSVNNDMIVTDNNGAVKFPQLCKFCDVRFSTCDNQKSCMSNCSITSICEKPQEVCVAVWRKNDENITLETVCHDPKLPYHDFILEDAASPKCIMKEKKKPGETFFMCSCSSDECNDNIIFSEEYNTSNPD

SEQ ID NO: 103 - protein, 500 aa, Artificial Sequence
  hIgG4FcdeltaK-CC-228P-T22d35 fusion
ESKYGPPCPPCPAPEFLGGPSVFLFPPKPKDTLMISRTPEVTCVVVDVSQEDPEVQFNWYVDGVEVHNAKTKPREEQFNSTYRVVSVLTVLHQDWLNGKEYKCKVSNKGLPSSIEKTISKAKGQPREPQVYTLPPSQEEMTKNQVSLTCLVKGFYPSDIAVEWESNGQPENNYKTTPPVLDSDGSFFLYSRLTVDKSRWQEGNVFSCSVMHEALHNHYTQKSLSLSLGIPPHVQKSVNNDMIVTDNNGAVKFPQLCKFCDVRFSTCDNQKSCMSNCSITSICEKPQEVCVAVWRKNDENITLETVCHDPKLPYHDFILEDAASPKCIMKEKKKPGETFFMCSCSSDECNDNIIFSEEYNTSNPDIPPHVQKSVNNDMIVTDNNGAVKFPQLCKFCDVRFSTCDNQKSCMSNCSITSICEKPQEVCVAVWRKNDENITLETVCHDPKLPYHDFILEDAASPKCIMKEKKKPGETFFMCSCSSDECNDNIIFSEEYNTSNPD

SEQ ID NO: 104 - protein, 500 aa, Artificial Sequence
  hIgG4FcdeltaK-CC-228P-409K-T22d35 fusion
ESKYGPPCPPCPAPEFLGGPSVFLFPPKPKDTLMISRTPEVTCVVVDVSQEDPEVQFNWYVDGVEVHNAKTKPREEQFNSTYRVVSVLTVLHQDWLNGKEYKCKVSNKGLPSSIEKTISKAKGQPREPQVYTLPPSQEEMTKNQVSLTCLVKGFYPSDIAVEWESNGQPENNYKTTPPVLDSDGSFFLYSKLTVDKSRWQEGNVFSCSVMHEALHNHYTQKSLSLSLGIPPHVQKSVNNDMIVTDNNGAVKFPQLCKFCDVRFSTCDNQKSCMSNCSITSICEKPQEVCVAVWRKNDENITLETVCHDPKLPYHDFILEDAASPKCIMKEKKKPGETFFMCSCSSDECNDNIIFSEEYNTSNPDIPPHVQKSVNNDMIVTDNNGAVKFPQLCKFCDVRFSTCDNQKSCMSNCSITSICEKPQEVCVAVWRKNDENITLETVCHDPKLPYHDFILEDAASPKCIMKEKKKPGETFFMCSCSSDECNDNIIFSEEYNTSNPD

SEQ ID NO: 105 - protein, 519 aa, Artificial Sequence
  hIgG2Fc-CCCC-T22d35 fusion, also termed Fc-T22d35
MDWTWRILFLVAAATGTHAERKCCVECPPCPAPPVAGPSVFLFPPKPKDTLMISRTPEVTCVVVDVSHEDPEVQFNWYVDGVEVHNAKTKPREEQFNSTFRVVSVLTVVHQDWLNGKEYKCKVSNKGLPAPIEKTISKTKGQPREPQVYTLPPSREEMTKNQVSLTCLVKGFYPSDISVEWESNGQPENNYKTTPPMLDSDGSFFLYSKLTVDKSRWQQGNVFSCSVMHEALHNHYTQKSLSLSPGKIPPHVQKSVNNDMIVTDNNGAVKFPQLCKFCDVRFSTCDNQKSCMSNCSITSICEKPQEVCVAVWRKNDENITLETVCHDPKLPYHDFILEDAASPKCIMKEKKKPGETFFMCSCSSDECNDNIIFSEEYNTSNPDIPPHVQKSVNNDMIVTDNNGAVKFPQLCKFCDVRFSTCDNQKSCMSNCSITSICEKPQEVCVAVWRKNDENITLETVCHDPKLPYHDFILEDAASPKCIMKEKKKPGETFFMCSCSSDECNDNIIFSEEYNTSNPD

SEQ ID NO: 106 - protein, 517 aa, Artificial Sequence
  hIgG1FcdeltaK-C-T2-T2bAA fusion
PPCPAPELLGGPSVFLFPPKPKDTLMISRTPEVTCVVVDVSHEDPEVKFNWYVDGVEVHNAKTKPREEQYNSTYRVVSVLTVLHQDWLNGKEYKCKVSNKALPAPIEKTISKAKGQPREPQVYTLPPSRDELTKNQVSLTCLVKGFYPSDIAVEWESNGQPENNYKTTPPVLDSDGSFFLYSKLTVDKSRWQQGNVFSCSVMHEALHNHYTQKSLSLSPGIPPHVQKSVNNDMIVTDNNGAVKFPQLCKFCDVRFSTCDNQKSCMSNCSITSICEKPQEVCVAVWRKNDENITLETVCHDPKLPYHDFILEDAASPKCIMKEKKKPGETFFMCSCSSDECNDNIIFSEEYNTSNPDIPPHVQKSDVEMEAQKDEIIAPSANRTAHPLRHINNDMIVTDNNGAVKFPQLCKFCDVRFSTCDNQKSCMSNCSITSICEKPQEVCVAVWRKNDENITLETVCHDPKLPYHDFILEDAASPKCIMKEKKKPGETFFMCSCSSDECNDNIIFSEEYNTSNPD

SEQ ID NO: 107 - protein, 523 aa, Artificial Sequence
  hIgG1FcdeltaK-CC-T2-T2bAA fusion
DKTHTCPPCPAPELLGGPSVFLFPPKPKDTLMISRTPEVTCVVVDVSHEDPEVKFNWYVDGVEVHNAKTKPREEQYNSTYRVVSVLTVLHQDWLNGKEYKCKVSNKALPAPIEKTISKAKGQPREPQVYTLPPSRDELTKNQVSLTCLVKGFYPSDIAVEWESNGQPENNYKTTPPVLDSDGSFFLYSKLTVDKSRWQQGNVFSCSVMHEALHNHYTQKSLSLSPGIPPHVQKSVNNDMIVTDNNGAVKFPQLCKFCDVRFSTCDNQKSCMSNCSITSICEKPQEVCVAVWRKNDENITLETVCHDPKLPYHDFILEDAASPKCIMKEKKKPGETFFMCSCSSDECNDNIIFSEEYNTSNPDIPPHVQKSDVEMEAQKDEIIAPSANRTAHPLRHINNDMIVTDNNGAVKFPQLCKFCDVRFSTCDNQKSCMSNCSITSICEKPQEVCVAVWRKNDENITLETVCHDPKLPYHDFILEDAASPKCIMKEKKKPGETFFMCSCSSDECNDNIIFSEEYNTSNPD

SEQ ID NO: 108 - protein, 519 aa, Artificial Sequence
  hIgG2FcdeltaK-CC-T2-T2bAA fusion
VECPPCPAPPVAGPSVFLFPPKPKDTLMISRTPEVTCVVVDVSHEDPEVQFNWYVDGVEVHNAKTKPREEQFNSTFRVVSVLTVVHQDWLNGKEYKCKVSNKGLPAPIEKTISKTKGQPREPQVYTLPPSREEMTKNQVSLTCLVKGFYPSDISVEWESNGQPENNYKTTPPMLDSDGSFFLYSKLTVDKSRWQQGNVFSCSVMHEALHNHYTQKSLSLSPGIPPHVQKSVNNDMIVTDNNGAVKFPQLCKFCDVRFSTCDNQKSCMSNCSITSICEKPQEVCVAVWRKNDENITLETVCHDPKLPYHDFILEDAASPKCIMKEKKKPGETFFMCSCSSDECNDNIIFSEEYNTSNPDIPPHVQKSDVEMEAQKDEIIAPSANRTAHPLRHINNDMIVTDNNGAVKFPQLCKFCDVRFSTCDNQKSCMSNCSITSICEKPQEVCVAVWRKNDENITLETVCHDPKLPYHDFILEDAASPKCIMKEKKKPGETFFMCSCSSDECNDNIIFSEEYNTSNPD

SEQ ID NO: 109 - protein, 525 aa, Artificial Sequence
  hIgG4FcdeltaK-CC-228P-T2-T2bAA fusion
ESKYGPPCPPCPAPEFLGGPSVFLFPPKPKDTLMISRTPEVTCVVVDVSQEDPEVQFNWYVDGVEVHNAKTKPREEQFNSTYRVVSVLTVLHQDWLNGKEYKCKVSNKGLPSSIEKTISKAKGQPREPQVYTLPPSQEEMTKNQVSLTCLVKGFYPSDIAVEWESNGQPENNYKTTPPVLDSDGSFFLYSRLTVDKSRWQEGNVFSCSVMHEALHNHYTQKSLSLSLGIPPHVQKSVNNDMIVTDNNGAVKFPQLCKFCDVRFSTCDNQKSCMSNCSITSICEKPQEVCVAVWRKNDENITLETVCHDPKLPYHDFILEDAASPKCIMKEKKKPGETFFMCSCSSDECNDNIIFSEEYNTSNPDIPPHVQKSDVEMEAQKDEIIAPSANRTAHPLRHINNDMIVTDNNGAVKFPQLCKFCDVRFSTCDNQKSCMSNCSITSICEKPQEVCVAVWRKNDENITLETVCHDPKLPYHDFILEDAASPKCIMKEKKKPGETFFMCSCSSDECNDNIIFSEEYNTSNPD

SEQ ID NO: 110 - protein, 525 aa, Artificial Sequence
  hIgG4FcdeltaK-CC-228P-409K-T2-T2bAA fusion
ESKYGPPCPPCPAPEFLGGPSVFLFPPKPKDTLMISRTPEVTCVVVDVSQEDPEVQFNWYVDGVEVHNAKTKPREEQFNSTYRVVSVLTVLHQDWLNGKEYKCKVSNKGLPSSIEKTISKAKGQPREPQVYTLPPSQEEMTKNQVSLTCLVKGFYPSDIAVEWESNGQPENNYKTTPPVLDSDGSFFLYSKLTVDKSRWQEGNVFSCSVMHEALHNHYTQKSLSLSLGIPPHVQKSVNNDMIVTDNNGAVKFPQLCKFCDVRFSTCDNQKSCMSNCSITSICEKPQEVCVAVWRKNDENITLETVCHDPKLPYHDFILEDAASPKCIMKEKKKPGETFFMCSCSSDECNDNIIFSEEYNTSNPDIPPHVQKSDVEMEAQKDEIIAPSANRTAHPLRHINNDMIVTDNNGAVKFPQLCKFCDVRFSTCDNQKSCMSNCSITSICEKPQEVCVAVWRKNDENITLETVCHDPKLPYHDFILEDAASPKCIMKEKKKPGETFFMCSCSSDECNDNIIFSEEYNTSNPD

SEQ ID NO: 111 - protein, 628 aa, Artificial Sequence
  hIgG1FcdeltaK-C-T2-T2-T2 fusion
PPCPAPELLGGPSVFLFPPKPKDTLMISRTPEVTCVVVDVSHEDPEVKFNWYVDGVEVHNAKTKPREEQYNSTYRVVSVLTVLHQDWLNGKEYKCKVSNKALPAPIEKTISKAKGQPREPQVYTLPPSRDELTKNQVSLTCLVKGFYPSDIAVEWESNGQPENNYKTTPPVLDSDGSFFLYSKLTVDKSRWQQGNVFSCSVMHEALHNHYTQKSLSLSPGIPPHVQKSVNNDMIVTDNNGAVKFPQLCKFCDVRFSTCDNQKSCMSNCSITSICEKPQEVCVAVWRKNDENITLETVCHDPKLPYHDFILEDAASPKCIMKEKKKPGETFFMCSCSSDECNDNIIFSEEYNTSNPDIPPHVQKSVNNDMIVTDNNGAVKFPQLCKFCDVRFSTCDNQKSCMSNCSITSICEKPQEVCVAVWRKNDENITLETVCHDPKLPYHDFILEDAASPKCIMKEKKKPGETFFMCSCSSDECNDNIIFSEEYNTSNPDIPPHVQKSVNNDMIVTDNNGAVKFPQLCKFCDVRFSTCDNQKSCMSNCSITSICEKPQEVCVAVWRKNDENITLETVCHDPKLPYHDFILEDAASPKCIMKEKKKPGETFFMCSCSSDECNDNIIFSEEYNTSNPD

SEQ ID NO: 112 - protein, 634 aa, Artificial Sequence
  hIgG1FcdeltaK-CC-T2-T2-T2 fusion
DKTHTCPPCPAPELLGGPSVFLFPPKPKDTLMISRTPEVTCVVVDVSHEDPEVKFNWYVDGVEVHNAKTKPREEQYNSTYRVVSVLTVLHQDWLNGKEYKCKVSNKALPAPIEKTISKAKGQPREPQVYTLPPSRDELTKNQVSLTCLVKGFYPSDIAVEWESNGQPENNYKTTPPVLDSDGSFFLYSKLTVDKSRWQQGNVFSCSVMHEALHNHYTQKSLSLSPGIPPHVQKSVNNDMIVTDNNGAVKFPQLCKFCDVRFSTCDNQKSCMSNCSITSICEKPQEVCVAVWRKNDENITLETVCHDPKLPYHDFILEDAASPKCIMKEKKKPGETFFMCSCSSDECNDNIIFSEEYNTSNPDIPPHVQKSVNNDMIVTDNNGAVKFPQLCKFCDVRFSTCDNQKSCMSNCSITSICEKPQEVCVAVWRKNDENITLETVCHDPKLPYHDFILEDAASPKCIMKEKKKPGETFFMCSCSSDECNDNIIFSEEYNTSNPDIPPHVQKSVNNDMIVTDNNGAVKFPQLCKFCDVRFSTCDNQKSCMSNCSITSICEKPQEVCVAVWRKNDENITLETVCHDPKLPYHDFILEDAASPKCIMKEKKKPGETFFMCSCSSDECNDNIIFSEEYNTSNPD

SEQ ID NO: 113 - protein, 630 aa, Artificial Sequence
  hIgG2FcdeltaK-CC-T2-T2-T2 fusion
VECPPCPAPPVAGPSVFLFPPKPKDTLMISRTPEVTCVVVDVSHEDPEVQFNWYVDGVEVHNAKTKPREEQFNSTFRVVSVLTVVHQDWLNGKEYKCKVSNKGLPAPIEKTISKTKGQPREPQVYTLPPSREEMTKNQVSLTCLVKGFYPSDISVEWESNGQPENNYKTTPPMLDSDGSFFLYSKLTVDKSRWQQGNVFSCSVMHEALHNHYTQKSLSLSPGIPPHVQKSVNNDMIVTDNNGAVKFPQLCKFCDVRFSTCDNQKSCMSNCSITSICEKPQEVCVAVWRKNDENITLETVCHDPKLPYHDFILEDAASPKCIMKEKKKPGETFFMCSCSSDECNDNIIFSEEYNTSNPDIPPHVQKSVNNDMIVTDNNGAVKFPQLCKFCDVRFSTCDNQKSCMSNCSITSICEKPQEVCVAVWRKNDENITLETVCHDPKLPYHDFILEDAASPKCIMKEKKKPGETFFMCSCSSDECNDNIIFSEEYNTSNPDIPPHVQKSVNNDMIVTDNNGAVKFPQLCKFCDVRFSTCDNQKSCMSNCSITSICEKPQEVCVAVWRKNDENITLETVCHDPKLPYHDFILEDAASPKCIMKEKKKPGETFFMCSCSSDECNDNIIFSEEYNTSNPD

SEQ ID NO: 114 - protein, 636 aa, Artificial Sequence
  hIgG4FcdeltaK-CC-228P-T2-T2-T2 fusion
ESKYGPPCPPCPAPEFLGGPSVFLFPPKPKDTLMISRTPEVTCVVVDVSQEDPEVQFNWYVDGVEVHNAKTKPREEQFNSTYRVVSVLTVLHQDWLNGKEYKCKVSNKGLPSSIEKTISKAKGQPREPQVYTLPPSQEEMTKNQVSLTCLVKGFYPSDIAVEWESNGQPENNYKTTPPVLDSDGSFFLYSRLTVDKSRWQEGNVFSCSVMHEALHNHYTQKSLSLSLGIPPHVQKSVNNDMIVTDNNGAVKFPQLCKFCDVRFSTCDNQKSCMSNCSITSICEKPQEVCVAVWRKNDENITLETVCHDPKLPYHDFILEDAASPKCIMKEKKKPGETFFMCSCSSDECNDNIIFSEEYNTSNPDIPPHVQKSVNNDMIVTDNNGAVKFPQLCKFCDVRFSTCDNQKSCMSNCSITSICEKPQEVCVAVWRKNDENITLETVCHDPKLPYHDFILEDAASPKCIMKEKKKPGETFFMCSCSSDECNDNIIFSEEYNTSNPDIPPHVQKSVNNDMIVTDNNGAVKFPQLCKFCDVRFSTCDNQKSCMSNCSITSICEKPQEVCVAVWRKNDENITLETVCHDPKLPYHDFILEDAASPKCIMKEKKKPGETFFMCSCSSDECNDNIIFSEEYNTSNPD

SEQ ID NO: 115 - protein, 636 aa, Artificial Sequence
  hIgG4FcdeltaK-CC-228P-409K-T2-T2-T2 fusion
ESKYGPPCPPCPAPEFLGGPSVFLFPPKPKDTLMISRTPEVTCVVVDVSQEDPEVQFNWYVDGVEVHNAKTKPREEQFNSTYRVVSVLTVLHQDWLNGKEYKCKVSNKGLPSSIEKTISKAKGQPREPQVYTLPPSQEEMTKNQVSLTCLVKGFYPSDIAVEWESNGQPENNYKTTPPVLDSDGSFFLYSKLTVDKSRWQEGNVFSCSVMHEALHNHYTQKSLSLSLGIPPHVQKSVNNDMIVTDNNGAVKFPQLCKFCDVRFSTCDNQKSCMSNCSITSICEKPQEVCVAVWRKNDENITLETVCHDPKLPYHDFILEDAASPKCIMKEKKKPGETFFMCSCSSDECNDNIIFSEEYNTSNPDIPPHVQKSVNNDMIVTDNNGAVKFPQLCKFCDVRFSTCDNQKSCMSNCSITSICEKPQEVCVAVWRKNDENITLETVCHDPKLPYHDFILEDAASPKCIMKEKKKPGETFFMCSCSSDECNDNIIFSEEYNTSNPDIPPHVQKSVNNDMIVTDNNGAVKFPQLCKFCDVRFSTCDNQKSCMSNCSITSICEKPQEVCVAVWRKNDENITLETVCHDPKLPYHDFILEDAASPKCIMKEKKKPGETFFMCSCSSDECNDNIIFSEEYNTSNPD

SEQ ID NO: 116 - protein, 678 aa, Artificial Sequence
  hIgG1FcdeltaK-C-T2-T2bAA-T2bAA fusion
PPCPAPELLGGPSVFLFPPKPKDTLMISRTPEVTCVVVDVSHEDPEVKFNWYVDGVEVHNAKTKPREEQYNSTYRVVSVLTVLHQDWLNGKEYKCKVSNKALPAPIEKTISKAKGQPREPQVYTLPPSRDELTKNQVSLTCLVKGFYPSDIAVEWESNGQPENNYKTTPPVLDSDGSFFLYSKLTVDKSRWQQGNVFSCSVMHEALHNHYTQKSLSLSPGIPPHVQKSVNNDMIVTDNNGAVKFPQLCKFCDVRFSTCDNQKSCMSNCSITSICEKPQEVCVAVWRKNDENITLETVCHDPKLPYHDFILEDAASPKCIMKEKKKPGETFFMCSCSSDECNDNIIFSEEYNTSNPDIPPHVQKSDVEMEAQKDEIIAPSANRTAHPLRHINNDMIVTDNNGAVKFPQLCKFCDVRFSTCDNQKSCMSNCSITSICEKPQEVCVAVWRKNDENITLETVCHDPKLPYHDFILEDAASPKCIMKEKKKPGETFFMCSCSSDECNDNIIFSEEYNTSNPDIPPHVQKSDVEMEAQKDEIIAPSANRTAHPLRHINNDMIVTDNNGAVKFPQLCKFCDVRFSTCDNQKSCMSNCSITSICEKPQEVCVAVWRKNDENITLETVCHDPKLPYHDFILEDAASPKCIMKEKKKPGETFFMCSCSSDECNDNIIFSEEYNTSNPD

SEQ ID NO: 117 - protein, 684 aa, Artificial Sequence
  hIgG1FcdeltaK-CC-T2-T2bAA-T2bAA fusion
DKTHTCPPCPAPELLGGPSVFLFPPKPKDTLMISRTPEVTCVVVDVSHEDPEVKFNWYVDGVEVHNAKTKPREEQYNSTYRVVSVLTVLHQDWLNGKEYKCKVSNKALPAPIEKTISKAKGQPREPQVYTLPPSRDELTKNQVSLTCLVKGFYPSDIAVEWESNGQPENNYKTTPPVLDSDGSFFLYSKLTVDKSRWQQGNVFSCSVMHEALHNHYTQKSLSLSPGIPPHVQKSVNNDMIVTDNNGAVKFPQLCKFCDVRFSTCDNQKSCMSNCSITSICEKPQEVCVAVWRKNDENITLETVCHDPKLPYHDFILEDAASPKCIMKEKKKPGETFFMCSCSSDECNDNIIFSEEYNTSNPDIPPHVQKSDVEMEAQKDEIIAPSANRTAHPLRHINNDMIVTDNNGAVKFPQLCKFCDVRFSTCDNQKSCMSNCSITSICEKPQEVCVAVWRKNDENITLETVCHDPKLPYHDFILEDAASPKCIMKEKKKPGETFFMCSCSSDECNDNIIFSEEYNTSNPDIPPHVQKSDVEMEAQKDEIIAPSANRTAHPLRHINNDMIVTDNNGAVKFPQLCKFCDVRFSTCDNQKSCMSNCSITSICEKPQEVCVAVWRKNDENITLETVCHDPKLPYHDFILEDAASPKCIMKEKKKPGETFFMCSCSSDECNDNIIFSEEYNTSNPD

SEQ ID NO: 118 - protein, 680 aa, Artificial Sequence
  hIgG2FcdeltaK-CC-T2-T2bAA-T2bAA fusion
VECPPCPAPPVAGPSVFLFPPKPKDTLMISRTPEVTCVVVDVSHEDPEVQFNWYVDGVEVHNAKTKPREEQFNSTFRVVSVLTVVHQDWLNGKEYKCKVSNKGLPAPIEKTISKTKGQPREPQVYTLPPSREEMTKNQVSLTCLVKGFYPSDISVEWESNGQPENNYKTTPPMLDSDGSFFLYSKLTVDKSRWQQGNVFSCSVMHEALHNHYTQKSLSLSPGIPPHVQKSVNNDMIVTDNNGAVKFPQLCKFCDVRFSTCDNQKSCMSNCSITSICEKPQEVCVAVWRKNDENITLETVCHDPKLPYHDFILEDAASPKCIMKEKKKPGETFFMCSCSSDECNDNIIFSEEYNTSNPDIPPHVQKSDVEMEAQKDEIIAPSANRTAHPLRHINNDMIVTDNNGAVKFPQLCKFCDVRFSTCDNQKSCMSNCSITSICEKPQEVCVAVWRKNDENITLETVCHDPKLPYHDFILEDAASPKCIMKEKKKPGETFFMCSCSSDECNDNIIFSEEYNTSNPDIPPHVQKSDVEMEAQKDEIIAPSANRTAHPLRHINNDMIVTDNNGAVKFPQLCKFCDVRFSTCDNQKSCMSNCSITSICEKPQEVCVAVWRKNDENITLETVCHDPKLPYHDFILEDAASPKCIMKEKKKPGETFFMCSCSSDECNDNIIFSEEYNTSNPD

SEQ ID NO: 119 - protein, 686 aa, Artificial Sequence
  hIgG4FcdeltaK-CC-228P-T2-T2bAA-T2bAA fusion
ESKYGPPCPPCPAPEFLGGPSVFLFPPKPKDTLMISRTPEVTCVVVDVSQEDPEVQFNWYVDGVEVHNAKTKPREEQFNSTYRVVSVLTVLHQDWLNGKEYKCKVSNKGLPSSIEKTISKAKGQPREPQVYTLPPSQEEMTKNQVSLTCLVKGFYPSDIAVEWESNGQPENNYKTTPPVLDSDGSFFLYSRLTVDKSRWQEGNVFSCSVMHEALHNHYTQKSLSLSLGIPPHVQKSVNNDMIVTDNNGAVKFPQLCKFCDVRFSTCDNQKSCMSNCSITSICEKPQEVCVAVWRKNDENITLETVCHDPKLPYHDFILEDAASPKCIMKEKKKPGETFFMCSCSSDECNDNIIFSEEYNTSNPDIPPHVQKSDVEMEAQKDEIIAPSANRTAHPLRHINNDMIVTDNNGAVKFPQLCKFCDVRFSTCDNQKSCMSNCSITSICEKPQEVCVAVWRKNDENITLETVCHDPKLPYHDFILEDAASPKCIMKEKKKPGETFFMCSCSSDECNDNIIFSEEYNTSNPDIPPHVQKSDVEMEAQKDEIIAPSANRTAHPLRHINNDMIVTDNNGAVKFPQLCKFCDVRFSTCDNQKSCMSNCSITSICEKPQEVCVAVWRKNDENITLETVCHDPKLPYHDFILEDAASPKCIMKEKKKPGETFFMCSCSSDECNDNIIFSEEYNTSNPD

SEQ ID NO: 120 - protein, 686 aa, Artificial Sequence
  hIgG4FcdeltaK-CC-228P-409K-T2-T2bAA-T2bAA fusion
ESKYGPPCPPCPAPEFLGGPSVFLFPPKPKDTLMISRTPEVTCVVVDVSQEDPEVQFNWYVDGVEVHNAKTKPREEQFNSTYRVVSVLTVLHQDWLNGKEYKCKVSNKGLPSSIEKTISKAKGQPREPQVYTLPPSQEEMTKNQVSLTCLVKGFYPSDIAVEWESNGQPENNYKTTPPVLDSDGSFFLYSKLTVDKSRWQEGNVFSCSVMHEALHNHYTQKSLSLSLGIPPHVQKSVNNDMIVTDNNGAVKFPQLCKFCDVRFSTCDNQKSCMSNCSITSICEKPQEVCVAVWRKNDENITLETVCHDPKLPYHDFILEDAASPKCIMKEKKKPGETFFMCSCSSDECNDNIIFSEEYNTSNPDIPPHVQKSDVEMEAQKDEIIAPSANRTAHPLRHINNDMIVTDNNGAVKFPQLCKFCDVRFSTCDNQKSCMSNCSITSICEKPQEVCVAVWRKNDENITLETVCHDPKLPYHDFILEDAASPKCIMKEKKKPGETFFMCSCSSDECNDNIIFSEEYNTSNPDIPPHVQKSDVEMEAQKDEIIAPSANRTAHPLRHINNDMIVTDNNGAVKFPQLCKFCDVRFSTCDNQKSCMSNCSITSICEKPQEVCVAVWRKNDENITLETVCHDPKLPYHDFILEDAASPKCIMKEKKKPGETFFMCSCSSDECNDNIIFSEEYNTSNPD

SEQ ID NO: 121 - protein, 214 aa, Artificial Sequence
  Cetuximab LC
DILLTQSPVILSVSPGERVSFSCRASQSIGTNIHWYQQRTNGSPRLLIKYASESISGIPSRFSGSGSGTDFTLSINSVESEDIADYYCQQNNNWPTTFGAGTKLELKRTVAAPSVFIFPPSDEQLKSGTASVVCLLNNFYPREAKVQWKVDNALQSGNSQESVTEQDSKDSTYSLSSTLTLSKADYEKHKVYACEVTHQGLSSPVTKSFNRGEC

SEQ ID NO: 122 - protein, 721 aa, Artificial Sequence
  Cetuximab HC-T22d35
QVQLKQSGPGLVQPSQSLSITCTVSGFSLTNYGVHWVRQSPGKGLEWLGVIWSGGNTDYNTPFTSRLSINKDNSKSQVFFKMNSLQSNDTAIYYCARALTYYDYEFAYWGQGTLVTVSAASTKGPSVFPLAPSSKSTSGGTAALGCLVKDYFPEPVTVSWNSGALTSGVHTFPAVLQSSGLYSLSSVVTVPSSSLGTQTYICNVNHKPSNTKVDKRVEPKSCDKTHTCPPCPAPELLGGPSVFLFPPKPKDTLMISRTPEVTCVVVDVSHEDPEVKFNWYVDGVEVHNAKTKPREEQYNSTYRVVSVLTVLHQDWLNGKEYKCKVSNKALPAPIEKTISKAKGQPREPQVYTLPPSRDELTKNQVSLTCLVKGFYPSDIAVEWESNGQPENNYKTTPPVLDSDGSFFLYSKLTVDKSRWQQGNVFSCSVMHEALHNHYTQKSLSLSPGKIPPHVQKSVNNDMIVTDNNGAVKFPQLCKFCDVRFSTCDNQKSCMSNCSITSICEKPQEVCVAVWRKNDENITLETVCHDPKLPYHDFILEDAASPKCIMKEKKKPGETFFMCSCSSDECNDNIIFSEEYNTSNPDIPPHVQKSVNNDMIVTDNNGAVKFPQLCKFCDVRFSTCDNQKSCMSNCSITSICEKPQEVCVAVWRKNDENITLETVCHDPKLPYHDFILEDAASPKCIMKEKKKPGETFFMCSCSSDECNDNIIFSEEYNTSNPD

SEQ ID NO: 123 - protein, 585 aa, Artificial Sequence
  Cetuximab HC-T2m
QVQLKQSGPGLVQPSQSLSITCTVSGFSLTNYGVHWVRQSPGKGLEWLGVIWSGGNTDYNTPFTSRLSINKDNSKSQVFFKMNSLQSNDTAIYYCARALTYYDYEFAYWGQGTLVTVSAASTKGPSVFPLAPSSKSTSGGTAALGCLVKDYFPEPVTVSWNSGALTSGVHTFPAVLQSSGLYSLSSVVTVPSSSLGTQTYICNVNHKPSNTKVDKRVEPKSCDKTHTCPPCPAPELLGGPSVFLFPPKPKDTLMISRTPEVTCVVVDVSHEDPEVKFNWYVDGVEVHNAKTKPREEQYNSTYRVVSVLTVLHQDWLNGKEYKCKVSNKALPAPIEKTISKAKGQPREPQVYTLPPSRDELTKNQVSLTCLVKGFYPSDIAVEWESNGQPENNYKTTPPVLDSDGSFFLYSKLTVDKSRWQQGNVFSCSVMHEALHNHYTQKSLSLSPGKIPPHVQKSVNNDMIVTDNNGAVKFPQLCKFCDVRFSTCDNQKSCMSNCSITSICEKPQEVCVAVWRKNDENITLETVCHDPKLPYHDFILEDAASPKCIMKEKKKPGETFFMCSCSSDECNDNIIFSEEYNTSNPD

SEQ ID NO: 124 - protein, 214 aa, Artificial Sequence
  Herceptin LC
DIQMTQSPSSLSASVGDRVTITCRASQDVNTAVAWYQQKPGKAPKLLIYSASFLYSGVPSRFSGSRSGTDFTLTISSLQPEDFATYYCQQHYTTPPTFGQGTKVEIKRTVAAPSVFIFPPSDEQLKSGTASVVCLLNNFYPREAKVQWKVDNALQSGNSQESVTEQDSKDSTYSLSSTLTLSKADYEKHKVYACEVTHQGLSSPVTKSFNRGEC

SEQ ID NO: 125 - protein, 722 aa, Artificial Sequence
  Herceptin HC-T22d35
EVQLVESGGGLVQPGGSLRLSCAASGFNIKDTYIHWVRQAPGKGLEWVARIYPTNGYTRYADSVKGRFTISADTSKNTAYLQMNSLRAEDTAVYYCSRWGGDGFYAMDYWGQGTLVTVSSASTKGPSVFPLAPSSKSTSGGTAALGCLVKDYFPEPVTVSWNSGALTSGVHTFPAVLQSSGLYSLSSVVTVPSSSLGTQTYICNVNHKPSNTKVDKKVEPKSCDKTHTCPPCPAPELLGGPSVFLFPPKPKDTLMISRTPEVTCVVVDVSHEDPEVKFNWYVDGVEVHNAKTKPREEQYNSTYRVVSVLTVLHQDWLNGKEYKCKVSNKALPAPIEKTISKAKGQPREPQVYTLPPSRDELTKNQVSLTCLVKGFYPSDIAVEWESNGQPENNYKTTPPVLDSDGSFFLYSKLTVDKSRWQQGNVFSCSVMHEALHNHYTQKSLSLSPGKIPPHVQKSVNNDMIVTDNNGAVKFPQLCKFCDVRFSTCDNQKSCMSNCSITSICEKPQEVCVAVWRKNDENITLETVCHDPKLPYHDFILEDAASPKCIMKEKKKPGETFFMCSCSSDECNDNIIFSEEYNTSNPDIPPHVQKSVNNDMIVTDNNGAVKFPQLCKFCDVRFSTCDNQKSCMSNCSITSICEKPQEVCVAVWRKNDENITLETVCHDPKLPYHDFILEDAASPKCIMKEKKKPGETFFMCSCSSDECNDNIIFSEEYNTSNPD

SEQ ID NO: 126 - protein, 214 aa, Artificial Sequence
  Avastin LC
DIQMTQSPSSLSASVGDRVTITCSASQDISNYLNWYQQKPGKAPKVLIYFTSSLHSGVPSRFSGSGSGTDFTLTISSLQPEDFATYYCQQYSTVPWTFGQGTKVEIKRTVAAPSVFIFPPSDEQLKSGTASVVCLLNNFYPREAKVQWKVDNALQSGNSQESVTEQDSKDSTYSLSSTLTLSKADYEKHKVYACEVTHQGLSSPVTKSFNRGEC

SEQ ID NO: 127 - protein, 725 aa, Artificial Sequence
  Avastin HC-T22d35
EVQLVESGGGLVQPGGSLRLSCAASGYTFTNYGMNWVRQAPGKGLEWVGWINTYTGEPTYAADFKRRFTFSLDTSKSTAYLQMNSLRAEDTAVYYCAKYPHYYGSSHWYFDVWGQGTLVTVSSASTKGPSVFPLAPSSKSTSGGTAALGCLVKDYFPEPVTVSWNSGALTSGVHTFPAVLQSSGLYSLSSVVTVPSSSLGTQTYICNVNHKPSNTKVDKKVEPKSCDKTHTCPPCPAPELLGGPSVFLFPPKPKDTLMISRTPEVTCVVVDVSHEDPEVKFNWYVDGVEVHNAKTKPREEQYNSTYRVVSVLTVLHQDWLNGKEYKCKVSNKALPAPIEKTISKAKGQPREPQVYTLPPSRDELTKNQVSLTCLVKGFYPSDIAVEWESNGQPENNYKTTPPVLDSDGSFFLYSKLTVDKSRWQQGNVFSCSVMHEALHNHYTQKSLSLSPGKIPPHVQKSVNNDMIVTDNNGAVKFPQLCKFCDVRFSTCDNQKSCMSNCSITSICEKPQEVCVAVWRKNDENITLETVCHDPKLPYHDFILEDAASPKCIMKEKKKPGETFFMCSCSSDECNDNIIFSEEYNTSNPDIPPHVQKSVNNDMIVTDNNGAVKFPQLCKFCDVRFSTCDNQKSCMSNCSITSICEKPQEVCVAVWRKNDENITLETVCHDPKLPYHDFILEDAASPKCIMKEKKKPGETFFMCSCSSDECNDNIIFSEEYNTSNPD

SEQ ID NO: 128 - protein, 213 aa, Artificial Sequence
  Synagis LC
DIQMTQSPSTLSASVGDRVTITCKCQLSVGYMHWYQQKPGKAPKLLIYDTSKLASGVPSRFSGSGSGTEFTLTISSLQPDDFATYYCFQGSGYPFTFGGGTKLEIKRTVAAPSVFIFPPSDEQLKSGTASVVCLLNNFYPREAKVQWKVDNALQSGNSQESVTEQDSKDSTYSLSSTLTLSKADYEKHKVYACEVTHQGLSSPVTKSFNRGEC

SEQ ID NO: 129 - protein, 721 aa, Artificial Sequence
  Synagis HC-T22d35
QVTLRESGPALVKPTQTLTLTCTFSGFSLSTSGMSVGWIRQPPGKALEWLADIWWDDKKDYNPSLKSRLTISKDTSKNQVVLKVTNMDPADTATYYCARSMITNWYFDVWGAGTTVTVSSASTKGPSVFPLAPSSAAAAGGTAALGCLVKDYFPEPVTVSWNSGALTSGVHTFPAVLQSSGLYSLSSVVTVPSSSLGTQTYICNVNHKPSNTKVDKRVEPKSCDKTHTCPPCPAPELLGGPSVFLFPPKPKDTLMISRTPEVTCVVVDVSHEDPEVKFNWYVDGVEVHNAKTKPREEQYNSTYRVVSVLTVLHQDWLNGKEYKCKVSNKALPAPIEKTISKAKGQPREPQVYTLPPSRDELTKNQVSLTCLVKGFYPSDIAVEWESNGQPENNYKTTPPVLDSDGSFFLYSKLTVDKSRWQQGNVFSCSVMHEALHNHYTQKSLSLSPGIPPHVQKSVNNDMIVTDNNGAVKFPQLCKFCDVRFSTCDNQKSCMSNCSITSICEKPQEVCVAVWRKNDENITLETVCHDPKLPYHDFILEDAASPKCIMKEKKKPGETFFMCSCSSDECNDNIIFSEEYNTSNPDIPPHVQKSVNNDMIVTDNNGAVKFPQLCKFCDVRFSTCDNQKSCMSNCSITSICEKPQEVCVAVWRKNDENITLETVCHDPKLPYHDFILEDAASPKCIMKEKKKPGETFFMCSCSSDECNDNIIFSEEYNTSNPD

SEQ ID NO: 130 - protein, 630 aa, Artificial Sequence
  FC5-Fc-T22d35
EVQLQASGGGLVQAGGSLRLSCAASGFKITHYTMGWFRQAPGKEREFVSRITWGGDNTFYSNSVKGRFTISRDNAKNTVYLQMNSLKPEDTADYYCAAGSTSTATPLRVDYWGKGTQVTVSSASEPRGPTIKPCPPCKCPAPNLLGGPSVFIFPPKIKDVLMISLSPIVTCVVVDVSEDDPDVQISWFVNNVEVHTAQTQTHREDYNSTLRVVSALPIQHQDWMSGKEFKCKVNNKDLPAPIERTISKPKGSVRAPQVYVLPPPEEEMTKKQVTLTCMVTDFMPEDIYVEWTNNGKTELNYKNTEPVLDSDGSYFMYSKLRVEKKNWVERNSYSCSVVHEGLHNHHTTKSFSRTPGTGIPPHVQKSVNNDMIVTDNNGAVKFPQLCKFCDVRFSTCDNQKSCMSNCSITSICEKPQEVCVAVWRKNDENITLETVCHDPKLPYHDFILEDAASPKCIMKEKKKPGETFFMCSCSSDECNDNIIFSEEYNTSNPDIPPHVQKSVNNDMIVTDNNGAVKFPQLCKFCDVRFSTCDNQKSCMSNCSITSICEKPQEVCVAVWRKNDENITLETVCHDPKLPYHDFILEDAASPKCIMKEKKKPGETFFMCSCSSDECNDNIIFSEEYNTSNPD

SEQ ID NO: 131 - protein, 494 aa, Artificial Sequence
  FC5-Fc-T2m
EVQLQASGGGLVQAGGSLRLSCAASGFKITHYTMGWFRQAPGKEREFVSRITWGGDNTFYSNSVKGRFTISRDNAKNTVYLQMNSLKPEDTADYYCAAGSTSTATPLRVDYWGKGTQVTVSSASEPRGPTIKPCPPCKCPAPNLLGGPSVFIFPPKIKDVLMISLSPIVTCVVVDVSEDDPDVQISWFVNNVEVHTAQTQTHREDYNSTLRVVSALPIQHQDWMSGKEFKCKVNNKDLPAPIERTISKPKGSVRAPQVYVLPPPEEEMTKKQVTLTCMVTDFMPEDIYVEWTNNGKTELNYKNTEPVLDSDGSYFMYSKLRVEKKNWVERNSYSCSVVHEGLHNHHTTKSFSRTPGTGIPPHVQKSVNNDMIVTDNNGAVKFPQLCKFCDVRFSTCDNQKSCMSNCSITSICEKPQEVCVAVWRKNDENITLETVCHDPKLPYHDFILEDAASPKCIMKEKKKPGETFFMCSCSSDECNDNIIFSEEYNTSNPD

SEQ ID NO: 132 - protein, 392 aa, Artificial Sequence
  T2-hIgG1Fc fusion from R&D, also termed T2m-Fc  (R&D)
MGRGLLRGLWPLHIVLWTRIASTIPPHVQKSVNNDMIVTDNNGAVKFPQLCKFCDVRFSTCDNQKSCMSNCSITSICEKPQEVCVAVWRKNDENITLETVCHDPKLPYHDFILEDAASPKCIMKEKKKPGETFFMCSCSSDECNDNIIFSEEYNTSNPDMDPKSCDKTHTCPPCPAPELLGGPSVFLFPPKPKDTLMISRTPEVTCVVVDVSHEDPEVKFNWYVDGVEVHNAKTKPREEQYNSTYRVVSVLTVLHQDWLNGKEYKCKVSNKALPAPIEKTISKAKGQPREPQVYTLPPSRDELTKNQVSLTCLVKGFYPSDIAVEWESNGQPENNYKTTPPVLDSDGSFFLYSKLTVDKSRWQQGNVFSCSVMHEALHNHYTQKSLSLSPGK

SEQ ID NO: 133 - protein, 382 aa, Artificial Sequence
  T2-hIgG2Fc-CCCC fusion, also termed T2m-Fc
MDWTWRILFLVAAATGTHAIPPHVQKSVNNDMIVTDNNGAVKFPQLCKFCDVRFSTCDNQKSCMSNCSITSICEKPQEVCVAVWRKNDENITLETVCHDPKLPYHDFILEDAASPKCIMKEKKKPGETFFMCSCSSDECNDNIIFSEEYNTSNPDERKCCVECPPCPAPPVAGPSVFLFPPKPKDTLMISRTPEVTCVVVDVSHEDPEVQFNWYVDGVEVHNAKTKPREEQFNSTFRVVSVLTVVHQDWLNGKEYKCKVSNKGLPAPIEKTISKTKGQPREPQVYTLPPSREEMTKNQVSLTCLVKGFYPSDISVEWESNGQPENNYKTTPPMLDSDGSFFLYSKLTVDKSRWQQGNVFSCSVMHEALHNHYTQKSLSLSPG

SEQ ID NO: 134 - protein, 15 aa, Artificial Sequence
  Isotope-labelled peptide for T22d35
LPYHDFILEDAASPK

SEQ ID NO: 135 - protein, 8 aa, Artificial Sequence
  Isotope-labelled peptide for Cetuximab
ALPAPIEK

SEQ ID NO: 136 - protein, 372 aa, Artificial Sequence
  D10-hIgG1FcdeltaK-CC-T2m fusion
DDDDDDDDDDDKTHTCPPCPAPELLGGPSVFLFPPKPKDTLMISRTPEVTCVVVDVSHEDPEVKFNWYVDGVEVHNAKTKPREEQYNSTYRVVSVLTVLHQDWLNGKEYKCKVSNKALPAPIEKTISKAKGQPREPQVYTLPPSRDELTKNQVSLTCLVKGFYPSDIAVEWESNGQPENNYKTTPPVLDSDGSFFLYSKLTVDKSRWQQGNVFSCSVMHEALHNHYTQKSLSLSPGIPPHVQKSVNNDMIVTDNNGAVKFPQLCKFCDVRFSTCDNQKSCMSNCSITSICEKPQEVCVAVWRKNDENITLETVCHDPKLPYHDFILEDAASPKCIMKEKKKPGETFFMCSCSSDECNDNIIFSEEYNTSNPD

SEQ ID NO: 137 - protein, 376 aa, Artificial Sequence
  D10-G3S-hIgG1FcdeltaK-CC-T2m fusion
DDDDDDDDDDGGGSDKTHTCPPCPAPELLGGPSVFLFPPKPKDTLMISRTPEVTCVVVDVSHEDPEVKFNWYVDGVEVHNAKTKPREEQYNSTYRVVSVLTVLHQDWLNGKEYKCKVSNKALPAPIEKTISKAKGQPREPQVYTLPPSRDELTKNQVSLTCLVKGFYPSDIAVEWESNGQPENNYKTTPPVLDSDGSFFLYSKLTVDKSRWQQGNVFSCSVMHEALHNHYTQKSLSLSPGIPPHVQKSVNNDMIVTDNNGAVKFPQLCKFCDVRFSTCDNQKSCMSNCSITSICEKPQEVCVAVWRKNDENITLETVCHDPKLPYHDFILEDAASPKCIMKEKKKPGETFFMCSCSSDECNDNIIFSEEYNTSNPD

SEQ ID NO: 138 - protein, 366 aa, Artificial Sequence
  D10-hIgG1FcdeltaK-C-T2m fusion
DDDDDDDDDDPPCPAPELLGGPSVFLFPPKPKDTLMISRTPEVTCVVVDVSHEDPEVKFNWYVDGVEVHNAKTKPREEQYNSTYRVVSVLTVLHQDWLNGKEYKCKVSNKALPAPIEKTISKAKGQPREPQVYTLPPSRDELTKNQVSLTCLVKGFYPSDIAVEWESNGQPENNYKTTPPVLDSDGSFFLYSKLTVDKSRWQQGNVFSCSVMHEALHNHYTQKSLSLSPGIPPHVQKSVNNDMIVTDNNGAVKFPQLCKFCDVRFSTCDNQKSCMSNCSITSICEKPQEVCVAVWRKNDENITLETVCHDPKLPYHDFILEDAASPKCIMKEKKKPGETFFMCSCSSDECNDNIIFSEEYNTSNPD

SEQ ID NO: 139 - protein, 374 aa, Artificial Sequence
  D10-(G3S)2-hIgG1FcdeltaK-C-T2m fusion
DDDDDDDDDDGGGSGGGSPPCPAPELLGGPSVFLFPPKPKDTLMISRTPEVTCVVVDVSHEDPEVKFNWYVDGVEVHNAKTKPREEQYNSTYRVVSVLTVLHQDWLNGKEYKCKVSNKALPAPIEKTISKAKGQPREPQVYTLPPSRDELTKNQVSLTCLVKGFYPSDIAVEWESNGQPENNYKTTPPVLDSDGSFFLYSKLTVDKSRWQQGNVFSCSVMHEALHNHYTQKSLSLSPGIPPHVQKSVNNDMIVTDNNGAVKFPQLCKFCDVRFSTCDNQKSCMSNCSITSICEKPQEVCVAVWRKNDENITLETVCHDPKLPYHDFILEDAASPKCIMKEKKKPGETFFMCSCSSDECNDNIIFSEEYNTSNPD

SEQ ID NO: 140 - protein, 368 aa, Artificial Sequence
  D10-hIgG2FcdeltaK-CC-T2m fusion
DDDDDDDDDDVECPPCPAPPVAGPSVFLFPPKPKDTLMISRTPEVTCVVVDVSHEDPEVQFNWYVDGVEVHNAKTKPREEQFNSTFRVVSVLTVVHQDWLNGKEYKCKVSNKGLPAPIEKTISKTKGQPREPQVYTLPPSREEMTKNQVSLTCLVKGFYPSDISVEWESNGQPENNYKTTPPMLDSDGSFFLYSKLTVDKSRWQQGNVFSCSVMHEALHNHYTQKSLSLSPGIPPHVQKSVNNDMIVTDNNGAVKFPQLCKFCDVRFSTCDNQKSCMSNCSITSICEKPQEVCVAVWRKNDENITLETVCHDPKLPYHDFILEDAASPKCIMKEKKKPGETFFMCSCSSDECNDNIIFSEEYNTSNPD

SEQ ID NO: 141 - protein, 374 aa, Artificial Sequence
  D10-hIgG4FcdeltaK-CC-228P-T2m fusion
DDDDDDDDDDESKYGPPCPPCPAPEFLGGPSVFLFPPKPKDTLMISRTPEVTCVVVDVSQEDPEVQFNWYVDGVEVHNAKTKPREEQFNSTYRVVSVLTVLHQDWLNGKEYKCKVSNKGLPSSIEKTISKAKGQPREPQVYTLPPSQEEMTKNQVSLTCLVKGFYPSDIAVEWESNGQPENNYKTTPPVLDSDGSFFLYSRLTVDKSRWQEGNVFSCSVMHEALHNHYTQKSLSLSLGIPPHVQKSVNNDMIVTDNNGAVKFPQLCKFCDVRFSTCDNQKSCMSNCSITSICEKPQEVCVAVWRKNDENITLETVCHDPKLPYHDFILEDAASPKCIMKEKKKPGETFFMCSCSSDECNDNIIFSEEYNTSNPD

SEQ ID NO: 142 - protein, 374 aa, Artificial Sequence
  D10-hIgG4FcdeltaK-CC-228P-409K-T2m fusion
DDDDDDDDDDESKYGPPCPPCPAPEFLGGPSVFLFPPKPKDTLMISRTPEVTCVVVDVSQEDPEVQFNWYVDGVEVHNAKTKPREEQFNSTYRVVSVLTVLHQDWLNGKEYKCKVSNKGLPSSIEKTISKAKGQPREPQVYTLPPSQEEMTKNQVSLTCLVKGFYPSDIAVEWESNGQPENNYKTTPPVLDSDGSFFLYSKLTVDKSRWQEGNVFSCSVMHEALHNHYTQKSLSLSLGIPPHVQKSVNNDMIVTDNNGAVKFPQLCKFCDVRFSTCDNQKSCMSNCSITSICEKPQEVCVAVWRKNDENITLETVCHDPKLPYHDFILEDAASPKCIMKEKKKPGETFFMCSCSSDECNDNIIFSEEYNTSNPD

SEQ ID NO: 143 - protein, 508 aa, Artificial Sequence
  D10-hIgG1FcdeltaK-CC-T22d35 fusion
DDDDDDDDDDDKTHTCPPCPAPELLGGPSVFLFPPKPKDTLMISRTPEVTCVVVDVSHEDPEVKFNWYVDGVEVHNAKTKPREEQYNSTYRVVSVLTVLHQDWLNGKEYKCKVSNKALPAPIEKTISKAKGQPREPQVYTLPPSRDELTKNQVSLTCLVKGFYPSDIAVEWESNGQPENNYKTTPPVLDSDGSFFLYSKLTVDKSRWQQGNVFSCSVMHEALHNHYTQKSLSLSPGIPPHVQKSVNNDMIVTDNNGAVKFPQLCKFCDVRFSTCDNQKSCMSNCSITSICEKPQEVCVAVWRKNDENITLETVCHDPKLPYHDFILEDAASPKCIMKEKKKPGETFFMCSCSSDECNDNIIFSEEYNTSNPDIPPHVQKSVNNDMIVTDNNGAVKFPQLCKFCDVRFSTCDNQKSCMSNCSITSICEKPQEVCVAVWRKNDENITLETVCHDPKLPYHDFILEDAASPKCIMKEKKKPGETFFMCSCSSDECNDNIIFSEEYNTSNPD

SEQ ID NO: 144 - protein, 504 aa, Artificial Sequence
  D10-hIgG2FcdeltaK-CC-T22d35 fusion
DDDDDDDDDDVECPPCPAPPVAGPSVFLFPPKPKDTLMISRTPEVTCVVVDVSHEDPEVQFNWYVDGVEVHNAKTKPREEQFNSTFRVVSVLTVVHQDWLNGKEYKCKVSNKGLPAPIEKTISKTKGQPREPQVYTLPPSREEMTKNQVSLTCLVKGFYPSDISVEWESNGQPENNYKTTPPMLDSDGSFFLYSKLTVDKSRWQQGNVFSCSVMHEALHNHYTQKSLSLSPGIPPHVQKSVNNDMIVTDNNGAVKFPQLCKFCDVRFSTCDNQKSCMSNCSITSICEKPQEVCVAVWRKNDENITLETVCHDPKLPYHDFILEDAASPKCIMKEKKKPGETFFMCSCSSDECNDNIIFSEEYNTSNPDIPPHVQKSVNNDMIVTDNNGAVKFPQLCKFCDVRFSTCDNQKSCMSNCSITSICEKPQEVCVAVWRKNDENITLETVCHDPKLPYHDFILEDAASPKCIMKEKKKPGETFFMCSCSSDECNDNIIFSEEYNTSNPD

SEQ ID NO: 145 - protein, 510 aa, Artificial Sequence
  D10-hIgG4FcdeltaK-CC-228P-T22d35 fusion
DDDDDDDDDDESKYGPPCPPCPAPEFLGGPSVFLFPPKPKDTLMISRTPEVTCVVVDVSQEDPEVQFNWYVDGVEVHNAKTKPREEQFNSTYRVVSVLTVLHQDWLNGKEYKCKVSNKGLPSSIEKTISKAKGQPREPQVYTLPPSQEEMTKNQVSLTCLVKGFYPSDIAVEWESNGQPENNYKTTPPVLDSDGSFFLYSRLTVDKSRWQEGNVFSCSVMHEALHNHYTQKSLSLSLGIPPHVQKSVNNDMIVTDNNGAVKFPQLCKFCDVRFSTCDNQKSCMSNCSITSICEKPQEVCVAVWRKNDENITLETVCHDPKLPYHDFILEDAASPKCIMKEKKKPGETFFMCSCSSDECNDNIIFSEEYNTSNPDIPPHVQKSVNNDMIVTDNNGAVKFPQLCKFCDVRFSTCDNQKSCMSNCSITSICEKPQEVCVAVWRKNDENITLETVCHDPKLPYHDFILEDAASPKCIMKEKKKPGETFFMCSCSSDECNDNIIFSEEYNTSNPD

SEQ ID NO: 146 - protein, 510 aa, Artificial Sequence
  D10-hIgG4FcdeltaK-CC-228P-409K-T22d35 fusion
DDDDDDDDDDESKYGPPCPPCPAPEFLGGPSVFLFPPKPKDTLMISRTPEVTCVVVDVSQEDPEVQFNWYVDGVEVHNAKTKPREEQFNSTYRVVSVLTVLHQDWLNGKEYKCKVSNKGLPSSIEKTISKAKGQPREPQVYTLPPSQEEMTKNQVSLTCLVKGFYPSDIAVEWESNGQPENNYKTTPPVLDSDGSFFLYSKLTVDKSRWQEGNVFSCSVMHEALHNHYTQKSLSLSLGIPPHVQKSVNNDMIVTDNNGAVKFPQLCKFCDVRFSTCDNQKSCMSNCSITSICEKPQEVCVAVWRKNDENITLETVCHDPKLPYHDFILEDAASPKCIMKEKKKPGETFFMCSCSSDECNDNIIFSEEYNTSNPDIPPHVQKSVNNDMIVTDNNGAVKFPQLCKFCDVRFSTCDNQKSCMSNCSITSICEKPQEVCVAVWRKNDENITLETVCHDPKLPYHDFILEDAASPKCIMKEKKKPGETFFMCSCSSDECNDNIIFSEEYNTSNPD

SEQ ID NO: 147 - protein, 644 aa, Artificial Sequence
  D10-hIgG1FcdeltaK-CC-T2-T2-T2 fusion
DDDDDDDDDDDKTHTCPPCPAPELLGGPSVFLFPPKPKDTLMISRTPEVTCVVVDVSHEDPEVKFNWYVDGVEVHNAKTKPREEQYNSTYRVVSVLTVLHQDWLNGKEYKCKVSNKALPAPIEKTISKAKGQPREPQVYTLPPSRDELTKNQVSLTCLVKGFYPSDIAVEWESNGQPENNYKTTPPVLDSDGSFFLYSKLTVDKSRWQQGNVFSCSVMHEALHNHYTQKSLSLSPGIPPHVQKSVNNDMIVTDNNGAVKFPQLCKFCDVRFSTCDNQKSCMSNCSITSICEKPQEVCVAVWRKNDENITLETVCHDPKLPYHDFILEDAASPKCIMKEKKKPGETFFMCSCSSDECNDNIIFSEEYNTSNPDIPPHVQKSVNNDMIVTDNNGAVKFPQLCKFCDVRFSTCDNQKSCMSNCSITSICEKPQEVCVAVWRKNDENITLETVCHDPKLPYHDFILEDAASPKCIMKEKKKPGETFFMCSCSSDECNDNIIFSEEYNTSNPDIPPHVQKSVNNDMIVTDNNGAVKFPQLCKFCDVRFSTCDNQKSCMSNCSITSICEKPQEVCVAVWRKNDENITLETVCHDPKLPYHDFILEDAASPKCIMKEKKKPGETFFMCSCSSDECNDNIIFSEEYNTSNPD

SEQ ID NO: 148 - protein, 640 aa, Artificial Sequence
  D10-hIgG2FcdeltaK-CC-T2-T2-T2 fusion
DDDDDDDDDDVECPPCPAPPVAGPSVFLFPPKPKDTLMISRTPEVTCVVVDVSHEDPEVQFNWYVDGVEVHNAKTKPREEQFNSTFRVVSVLTVVHQDWLNGKEYKCKVSNKGLPAPIEKTISKTKGQPREPQVYTLPPSREEMTKNQVSLTCLVKGFYPSDISVEWESNGQPENNYKTTPPMLDSDGSFFLYSKLTVDKSRWQQGNVFSCSVMHEALHNHYTQKSLSLSPGIPPHVQKSVNNDMIVTDNNGAVKFPQLCKFCDVRFSTCDNQKSCMSNCSITSICEKPQEVCVAVWRKNDENITLETVCHDPKLPYHDFILEDAASPKCIMKEKKKPGETFFMCSCSSDECNDNIIFSEEYNTSNPDIPPHVQKSVNNDMIVTDNNGAVKFPQLCKFCDVRFSTCDNQKSCMSNCSITSICEKPQEVCVAVWRKNDENITLETVCHDPKLPYHDFILEDAASPKCIMKEKKKPGETFFMCSCSSDECNDNIIFSEEYNTSNPDIPPHVQKSVNNDMIVTDNNGAVKFPQLCKFCDVRFSTCDNQKSCMSNCSITSICEKPQEVCVAVWRKNDENITLETVCHDPKLPYHDFILEDAASPKCIMKEKKKPGETFFMCSCSSDECNDNIIFSEEYNTSNPD

SEQ ID NO: 149 - protein, 646 aa, Artificial Sequence
  D10-hIgG4FcdeltaK-CC-228P-T2-T2-T2 fusion
DDDDDDDDDDESKYGPPCPPCPAPEFLGGPSVFLFPPKPKDTLMISRTPEVTCVVVDVSQEDPEVQFNWYVDGVEVHNAKTKPREEQFNSTYRVVSVLTVLHQDWLNGKEYKCKVSNKGLPSSIEKTISKAKGQPREPQVYTLPPSQEEMTKNQVSLTCLVKGFYPSDIAVEWESNGQPENNYKTTPPVLDSDGSFFLYSRLTVDKSRWQEGNVFSCSVMHEALHNHYTQKSLSLSLGIPPHVQKSVNNDMIVTDNNGAVKFPQLCKFCDVRFSTCDNQKSCMSNCSITSICEKPQEVCVAVWRKNDENITLETVCHDPKLPYHDFILEDAASPKCIMKEKKKPGETFFMCSCSSDECNDNIIFSEEYNTSNPDIPPHVQKSVNNDMIVTDNNGAVKFPQLCKFCDVRFSTCDNQKSCMSNCSITSICEKPQEVCVAVWRKNDENITLETVCHDPKLPYHDFILEDAASPKCIMKEKKKPGETFFMCSCSSDECNDNIIFSEEYNTSNPDIPPHVQKSVNNDMIVTDNNGAVKFPQLCKFCDVRFSTCDNQKSCMSNCSITSICEKPQEVCVAVWRKNDENITLETVCHDPKLPYHDFILEDAASPKCIMKEKKKPGETFFMCSCSSDECNDNIIFSEEYNTSNPD

SEQ ID NO: 150 - protein, 649 aa, Artificial Sequence
  D10-hIgG4FcdeltaK-CC-228P-409K-T2-T2-T2 fusion
DDDDDDDDDDESKYGPPCPPCPAPEFLGGPSVFLFPPKPKDTLMISRTPEVTCVVVDVSQEDPEVQFNWYVDGVEVHNAKTKPREEQFNSTYRVVSVLTVLHQDWLNGKEYKCKVSNKGLPSSISEQEKTISKAKGQPREPQVYTLPPSQEEMTKNQVSLTCLVKGFYPSDIAVEWESNGQPENNYKTTPPVLDSDGSFFLYSKLTVDKSRWQEGNVFSCSVMHEALHNHYTQKSLSLSLGIPPHVQKSVNNDMIVTDNNGAVKFPQLCKFCDVRFSTCDNQKSCMSNCSITSICEKPQEVCVAVWRKNDENITLETVCHDPKLPYHDFILEDAASPKCIMKEKKKPGETFFMCSCSSDECNDNIIFSEEYNTSNPDIPPHVQKSVNNDMIVTDNNGAVKFPQLCKFCDVRFSTCDNQKSCMSNCSITSICEKPQEVCVAVWRKNDENITLETVCHDPKLPYHDFILEDAASPKCIMKEKKKPGETFFMCSCSSDECNDNIIFSEEYNTSNPDIPPHVQKSVNNDMIVTDNNGAVKFPQLCKFCDVRFSTCDNQKSCMSNCSITSICEKPQEVCVAVWRKNDENITLETVCHDPKLPYHDFILEDAASPKCIMKEKKKPGETFFMCSCSSDECNDNIIFSEEYNTSNPD